European Patent Application EP 4 530 359 A1, published April 2, 2025. Title: Multiplexed single molecule RNA FISH using DNA nanostructures. Applicant: Ludwig-Maximilians-Universität München. Application EP. The sequence listing filed with the application follows.

SEQUENCE LISTING (490 sequences)

SEQ ID NO: 1 - DNA, 28 bp, synthetic construct
  source 1..28: mol_type = other DNA
ttaaatcgctgctcggctgactctggtc

SEQ ID NO: 2 - DNA, 28 bp, synthetic construct
  source 1..28: mol_type = other DNA
gcgttttcagaacgaaagaggggttatc

SEQ ID NO: 3 - DNA, 28 bp, synthetic construct
  source 1..28: mol_type = other DNA
gtaccttaacgtcaaacaaccccatcaa

SEQ ID NO: 4 - DNA, 28 bp, synthetic construct
  source 1..28: mol_type = other DNA
tgctttgacgtaaaccgtaataaatttt

SEQ ID NO: 5 - DNA, 35 bp, synthetic construct
  source 1..35: mol_type = other DNA
aaatctaaaaccacttaatttctagcataaggcta

SEQ ID NO: 6 - DNA, 35 bp, synthetic construct
  source 1..35: mol_type = other DNA
ttaagaatcagatgaacaattgccccaaaaattaa

SEQ ID NO: 7 - DNA, 49 bp, synthetic construct
  source 1..49: mol_type = other DNA
gagcctatgtactgaatcctcattaaagcctcagacaagccggtcctga

SEQ ID NO: 8 - DNA, 49 bp, synthetic construct
  source 1..49: mol_type = other DNA
gaacaaggccgccaggtcatagccccctagcaaaagtaccgattataca

SEQ ID NO: 9 - DNA, 49 bp, synthetic construct
  source 1..49: mol_type = other DNA
attttatcagtgccgaggcaggtcagaccaccctcagaacggatgtaga

SEQ ID NO: 10 - DNA, 49 bp, synthetic construct; identical to SEQ ID NO: 9
  source 1..49: mol_type = other DNA

SEQ ID NO: 11 - DNA, 56 bp, synthetic construct
  source 1..56: mol_type = other DNA
agcaacgacagcttatattactccatcatgctgaatataatgaagtacgtagtagt

SEQ ID NO: 12 - DNA, 56 bp, synthetic construct
  source 1..56: mol_type = other DNA
atcgtcatcgcccagaagaacagtaatattttgataagaggtcccaattcatttgg

SEQ ID NO: 13 - DNA, 28 bp, synthetic construct
  source 1..28: mol_type = other DNA
attaacaaaacatcacgggtaaggcttt

SEQ ID NO: 14 - DNA, 28 bp, synthetic construct
  source 1..28: mol_type = other DNA
aaatgaattgaatgaacgaaacagcgaa

SEQ ID NO: 15 - DNA, 35 bp, synthetic construct
  source 1..35: mol_type = other DNA
agattttagcggaagacgttggaataaggaggttt

SEQ ID NO: 16 - DNA, 35 bp, synthetic construct
  source 1..35: mol_type = other DNA
tcaaaatttcatcataccttaaattgggtctaaga

SEQ ID NO: 17 - DNA, 35 bp, synthetic construct
  source 1..35: mol_type = other DNA
tttgcgtattgggcgtcgggaccgttctgagaaag

SEQ ID NO: 18 - DNA, 35 bp, synthetic construct
  source 1..35: mol_type = other DNA
agacgggcaacagcctaactcttgagagatgcaat

SEQ ID NO: 19 - DNA, 42 bp, synthetic construct
  source 1..42: mol_type = other DNA
agagtccactattatcccttattaaaataagattgtattaga

SEQ ID NO: 20 - DNA, 42 bp, synthetic construct
  source 1..42: mol_type = other DNA
gaaaaaccgtctataggcgaaaaccaatatatgtattgcccg

SEQ ID NO: 21 - DNA, 42 bp, synthetic construct
  source 1..42: mol_type = other DNA
accaagtaccctcacgcgttttcatcggattaccaccagtaa

SEQ ID NO: 22 - DNA, 42 bp, synthetic construct
  source 1..42: mol_type = other DNA
tttcatcaccggaagtttgccatcttttagccattattctgt

SEQ ID NO: 23 - DNA, 28 bp, synthetic construct
  source 1..28: mol_type = other DNA
aaaacatattttaaatctacagtcaatc

SEQ ID NO: 24 - DNA, 28 bp, synthetic construct
  source 1..28: mol_type = other DNA
agcaataaaagggtagctgataaacagg

SEQ ID NO: 25 - DNA, 35 bp, synthetic construct
  source 1..35: mol_type = other DNA
acaaccaccctcaggaggcaagtatcatataggct

SEQ ID NO: 26 - DNA, 35 bp, synthetic construct
  source 1..35: mol_type = other DNA
atccaatcgcaagatttagttaacagtagaggcat

SEQ ID NO: 27 - DNA, 35 bp, synthetic construct
  source 1..35: mol_type = other DNA
ttcttaagctacagaaatacgccatgttaactttg

SEQ ID NO: 28 - DNA, 35 bp, synthetic construct
  source 1..35: mol_type = other DNA
agttacaaaccctcggcatagtaagagctgtgaat

SEQ ID NO: 29 - DNA, 35 bp, synthetic construct
  source 1..35: mol_type = other DNA
gcttaggttgggttataccgaatatgcgcaaaagg

SEQ ID NO: 30 - DNA, 35 bp, synthetic construct
  source 1..35: mol_type = other DNA
gggagaaaggctttcattcaactaatgccagtcag

SEQ ID NO: 31 - DNA, 56 bp, synthetic construct
  source 1..56: mol_type = other DNA
cttagtggcaactactgtagcagtaaaagagtctgcgccagctggcagaagcccta

SEQ ID NO: 32 - DNA, 56 bp, synthetic construct
  source 1..56: mol_type = other DNA
tcttctagttgattcatttttatacttctttgatttcaaacttctggccaatattt

SEQ ID NO: 33 - DNA, 28 bp, synthetic construct
  source 1..28: mol_type = other DNA
gtaagaatgaacctaccctcattgagta

SEQ ID NO: 34 - DNA, 28 bp, synthetic construct
  source 1..28: mol_type = other DNA
gtctttatgagagcaaggaattcgtatt

SEQ ID NO: 35 - DNA, 28 bp, synthetic construct
  source 1..28: mol_type = other DNA
aaaatacgtgaggcaacaacttgaggat

SEQ ID NO: 36 - DNA, 35 bp, synthetic construct
  source 1..35: mol_type = other DNA
taacctgacttttgaaattttattgcctcggtaat

SEQ ID NO: 37 - DNA, 35 bp, synthetic construct
  source 1..35: mol_type = other DNA
aggtggcaaagctataatgtggagggtatgataat

SEQ ID NO: 38 - DNA, 35 bp, synthetic construct
  source 1..35: mol_type = other DNA
tatagccggattaggattagcacaggagatttgcc

SEQ ID NO: 39 - DNA, 35 bp, synthetic construct
  source 1..35: mol_type = other DNA
gaagtttaggcgcacataaggtggtttataatcat

SEQ ID NO: 40 - DNA, 35 bp, synthetic construct
  source 1..35: mol_type = other DNA
ataaatcggcaaagacagtcaaatatgaaaatatt

SEQ ID NO: 41 - DNA, 42 bp, synthetic construct
  source 1..42: mol_type = other DNA
tatatgtaaatgctacctaaaaccagtataagagaaaataat

SEQ ID NO: 42 - DNA, 42 bp, synthetic construct
  source 1..42: mol_type = other DNA
agagcggggaggccttataatcagtgagaaacgcttctgaaa

SEQ ID NO: 43 - DNA, 42 bp, synthetic construct
  source 1..42: mol_type = other DNA
cgcgagaaattctggaattacatcgccacgccaaccaataat

SEQ ID NO: 44 - DNA, 49 bp, synthetic construct
  source 1..49: mol_type = other DNA
tagaaaatcttctggatgcaatccaaaaaaaaggcatagttgatcggaa

SEQ ID NO: 45 - DNA, 49 bp, synthetic construct
  source 1..49: mol_type = other DNA
agtaaattatgggaactaaaggaattgcccgatatgccgcttacactca

SEQ ID NO: 46 - DNA, 49 bp, synthetic construct
  source 1..49: mol_type = other DNA
acgcaaaataaataacctccgttatcagctcgatacatagtgaaagact

SEQ ID NO: 47 - DNA, 56 bp, synthetic construct
  source 1..56: mol_type = other DNA
ttgaaaagcttagaagactacctttttaaggcgttagaaaaaccagacgaacgcgc

SEQ ID NO: 48 - DNA, 28 bp, synthetic construct
  source 1..28: mol_type = other DNA
ctgattactggctcgaaacacagcgaac

SEQ ID NO: 49 - DNA, 28 bp, synthetic construct
  source 1..28: mol_type = other DNA
aacaaagcgttaattaacaaaaagatta

SEQ ID NO: 50 - DNA, 35 bp, synthetic construct
  source 1..35: mol_type = other DNA
gcctaatccacacaacatacgctgacgcctgtaat

SEQ ID NO: 51 - DNA, 35 bp, synthetic construct
  source 1..35: mol_type = other DNA
ctgcccgtcatagctgtttccctggttgagagcat

SEQ ID NO: 52 - DNA, 35 bp, synthetic construct
  source 1..35: mol_type = other DNA
taccgcctgaaacatgaaagttgagtaacctgaat

SEQ ID NO: 53 - DNA, 49 bp, synthetic construct
  source 1..49: mol_type = other DNA
caacgtcgtggttctgttaaacagaaaacgacaactgaggaaacagatg

SEQ ID NO: 54 - DNA, 49 bp, synthetic construct
  source 1..49: mol_type = other DNA
catgcgcgaagtttgcttaatcgcaaattaaccgttaatatcgaccagt

SEQ ID NO: 55 - DNA, 49 bp, synthetic construct
  source 1..49: mol_type = other DNA
aggagaacgagtagttgctccacatcactttcgcgaaatagcccttctg

SEQ ID NO: 56 - DNA, 49 bp, synthetic construct
  source 1..49: mol_type = other DNA
cgaaatctggtttttcttttcgcgctcatgccggataggtaagccacgc

SEQ ID NO: 57 - DNA, 49 bp, synthetic construct
  source 1..49: mol_type = other DNA
actacgttccacgcaaataatcgtaaaataaaagtatcaatacttcatc

SEQ ID NO: 58 - DNA, 49 bp, synthetic construct
  source 1..49: mol_type = other DNA
tggtttgccttcaccgcctggctggggttcaggtctagaaccaccttgc

SEQ ID NO: 59 - DNA, 49 bp, synthetic construct
  source 1..49: mol_type = other DNA
agccaccgtaggaactgtttacggaacgccattaagccattatggatta

SEQ ID NO: 60 - DNA, 49 bp, synthetic construct
  source 1..49: mol_type = other DNA
aaccgccaccgcacatcccattaaattgaacctaagctattaaataaaa

SEQ ID NO: 61 - DNA, 56 bp, synthetic construct
  source 1..56: mol_type = other DNA
cgtcgagtgctcagtaccaggtcatacacagccatccggtatcttgagagaaccga

SEQ ID NO: 62 - DNA, 56 bp, synthetic construct
  source 1..56: mol_type = other DNA
caccgtaggctgagactcctcgttttaacgagcgtcttgcgggcttgcctacagac

SEQ ID NO: 63 - DNA, 40 bp, synthetic construct
  source 1..40: mol_type = other DNA
ccccgctttatgacaatgtcccgaaaaaaaaccaaaataa

SEQ ID NO: 64 - DNA, 35 bp, synthetic construct
  source 1..35: mol_type = other DNA
cagcgccaatatatcaaagaaaattttttcacgtt

SEQ ID NO: 65 - DNA, 35 bp, synthetic construct
  source 1..35: mol_type = other DNA
ctcaggaggtttagaagtcaggagaattatttagg

SEQ ID NO: 66 - DNA, 35 bp, synthetic construct
  source 1..35: mol_type = other DNA
agtttatgtttgaaatataacggagcctttaattg

SEQ ID NO: 67 - DNA, 35 bp, synthetic construct
  source 1..35: mol_type = other DNA
agggttgatataagacaagaatacagagaaaagga

SEQ ID NO: 68 - DNA, 42 bp, synthetic construct
  source 1..42: mol_type = other DNA
acctgcttaatgccaactgatttcaccactactaagtgtctg

SEQ ID NO: 69 - DNA, 42 bp, synthetic construct
  source 1..42: mol_type = other DNA
caacagtagattcaaagcctcgtgtaatgactctatgatacc

SEQ ID NO: 70 - DNA, 42 bp, synthetic construct
  source 1..42: mol_type = other DNA
gagatttaagaatacacagacaacagagatattttctgcgaa

SEQ ID NO: 71 - DNA, 42 bp, synthetic construct
  source 1..42: mol_type = other DNA
aagcatcctcatattatgaccatttcacactcgtcggtgggc

SEQ ID NO: 72 - DNA, 35 bp, synthetic construct
  source 1..35: mol_type = other DNA
agcgcatacgctaacggggtccttgatattcacaa

SEQ ID NO: 73 - DNA, 35 bp, synthetic construct
  source 1..35: mol_type = other DNA
aaaatagaaataaatggctttggaaagcgcagtct

SEQ ID NO: 74 - DNA, 42 bp, synthetic construct
  source 1..42: mol_type = other DNA
tagtatcccgtgtggacaccacggaatagtgaatttagagcc

SEQ ID NO: 75 - DNA, 42 bp, synthetic construct
  source 1..42: mol_type = other DNA
aacgctcaatttcattcatatggtttacgagggagggccgga

SEQ ID NO: 76 - DNA, 42 bp, synthetic construct
  source 1..42: mol_type = other DNA
tctttagactgaccacttagctcaacaataaagtatgggaat

SEQ ID NO: 77 - DNA, 49 bp, synthetic construct
  source 1..49: mol_type = other DNA
cagggctaaaattaagcattatttacatcattgcaggtgaattatcggt

SEQ ID NO: 78 - DNA, 49 bp, synthetic construct
  source 1..49: mol_type = other DNA
atttctctgtaccaggcgcgagggacatatcggccaatgacagaaaatc

SEQ ID NO: 79 - DNA, 56 bp, synthetic construct
  source 1..56: mol_type = other DNA
aaatcaacaggcgccgcctgacctaatttttcgagttagcaaggaaggtaaatatt

SEQ ID NO: 80 - DNA, 23 bp, synthetic construct
  source 1..23: mol_type = other DNA
aaaagtacgccagaatcctgaga

SEQ ID NO: 81 - DNA, 23 bp, synthetic construct
  source 1..23: mol_type = other DNA
aaaaaagggaagaaagcgaaagg

SEQ ID NO: 82 - DNA, 23 bp, synthetic construct
  source 1..23: mol_type = other DNA
aaaaagatgatgaaacaaacatc

SEQ ID NO: 83 - DNA, 23 bp, synthetic construct
  source 1..23: mol_type = other DNA
aaaaaagcaaactccaacaggtc

SEQ ID NO: 84 - DNA, 23 bp, synthetic construct
  source 1..23: mol_type = other DNA
aaaacgccattcgccattcaggc

SEQ ID NO: 85 - DNA, 23 bp, synthetic construct
  source 1..23: mol_type = other DNA
aaaagccctttttaagaaaagta

SEQ ID NO: 86 - DNA, 23 bp, synthetic construct
  source 1..23: mol_type = other DNA
aaaagaatttatcaaaatcatag

SEQ ID NO: 87 - DNA, 23 bp, synthetic construct
  source 1..23: mol_type = other DNA
aaaacagcggagtgagaatagaa

SEQ ID NO: 88 - DNA, 23 bp, synthetic construct
  source 1..23: mol_type = other DNA
aaaaccaccaccctcattttcag

SEQ ID NO: 89 - DNA, 23 bp, synthetic construct
  source 1..23: mol_type = other DNA
aaaaactgcggaatcgtcataaa

SEQ ID NO: 90 - DNA, 34 bp, synthetic construct
  source 1..34: mol_type = other DNA
ttttgaaactacaacgcctaaaaaaaagtagcat

SEQ ID NO: 91 - DNA, 34 bp, synthetic construct
  source 1..34: mol_type = other DNA
atggttgaaaaaaaactttgacgagcacgggcaa

SEQ ID NO: 92 - DNA, 34 bp, synthetic construct
  source 1..34: mol_type = other DNA
atttcaacagtacataaataaaaaaaacaatata

SEQ ID NO: 93 - DNA, 34 bp, synthetic construct
  source 1..34: mol_type = other DNA
taccgatacccaaaagaacaaaaaaaatggcatg

SEQ ID NO: 94 - DNA, 39 bp, synthetic construct
  source 1..39: mol_type = other DNA
tcatttgaattaaaaaaaaaccttttttaatggaaactt

SEQ ID NO: 95 - DNA, 39 bp, synthetic construct
  source 1..39: mol_type = other DNA
aaccgaggaaacaaaaaaaagcaataataacggattcca

SEQ ID NO: 96 - DNA, 39 bp, synthetic construct
  source 1..39: mol_type = other DNA
ggcctcttcgctaaaaaaaaattacgccagctggtgcag

SEQ ID NO: 97 - DNA, 39 bp, synthetic construct
  source 1..39: mol_type = other DNA
agagtcgaaagggggatgtaaaaaaaagctgcaaggcga

SEQ ID NO: 98 - DNA, 39 bp, synthetic construct
  source 1..39: mol_type = other DNA
atacatataacgtgctttcaaaaaaaactcgttagaatc

SEQ ID NO: 99 - DNA, 39 bp, synthetic construct
  source 1..39: mol_type = other DNA
gtaacactgagtaaaaaaaattcgtcaccagtaccaccc

SEQ ID NO: 100 - DNA, 40 bp, synthetic construct
  source 1..40: mol_type = other DNA
tcaatcgcatggaaatacctacaaaaaaaaattttgacgc

SEQ ID NO: 101 - DNA, 40 bp, synthetic construct
  source 1..40: mol_type = other DNA
cctgtagccaaaaaaaaagctttcatcaacatttggcctt

SEQ ID NO: 102 - DNA, 40 bp, synthetic construct
  source 1..40: mol_type = other DNA
caagaaccgaaaaaaaagatattcattacccaaatcttga

SEQ ID NO: 103 - DNA, 40 bp, synthetic construct
  source 1..40: mol_type = other DNA
ttttgttatcccaatccaaataaaaaaaaaagaaacgatt

SEQ ID NO: 104 - DNA, 40 bp, synthetic construct
  source 1..40: mol_type = other DNA
ttagatacaaaaaaaaatttcgcaaatggtcaattgacca

SEQ ID NO: 105 - DNA, 40 bp, synthetic construct
  source 1..40: mol_type = other DNA
tccagttagcccgagatagggttaaaaaaaagagtgttgt

SEQ ID NO: 106 - DNA, 40 bp, synthetic construct
  source 1..40: mol_type = other DNA
cgctgaggcaaaaaaaattgcagggagttaaagattcggt

SEQ ID NO: 107 - DNA, 40 bp, synthetic construct
  source 1..40: mol_type = other DNA
agcctttataaaaaaaattcaacgcaaggataacgggaga

SEQ ID NO: 108 - DNA, 40 bp, synthetic construct
  source 1..40: mol_type = other DNA
aacagagcgaacgaaccaccagcaaaaaaaaagaagataa

SEQ ID NO: 109 - DNA, 40 bp, synthetic construct
  source 1..40: mol_type = other DNA
gaacaacataaaaaaaatattacaggtagaaagactaacg

SEQ ID NO: 110 - DNA, 40 bp, synthetic construct
  source 1..40: mol_type = other DNA
gaagggtgtttggattatacttcaaaaaaaatgaataatg

SEQ ID NO: 111 - DNA, 40 bp, synthetic construct
  source 1..40: mol_type = other DNA
tatagaacgcgcccaatagcaagaaaaaaaacaaatcaga

SEQ ID NO: 112 - DNA, 40 bp, synthetic construct
  source 1..40: mol_type = other DNA
aattactaaataagaataaacacaaaaaaaacggaatcat

SEQ ID NO: 113 - DNA, 40 bp, synthetic construct
  source 1..40: mol_type = other DNA
ggaacctacagttaatgccccctaaaaaaaagcctatttc

SEQ ID NO: 114 - DNA, 40 bp, synthetic construct
  source 1..40: mol_type = other DNA
atccccgcttgttacctcgataaaaaaaaaaagacggagg

SEQ ID NO: 115 - DNA, 40 bp, synthetic construct
  source 1..40: mol_type = other DNA
gcggggagctgcattaatgaatcaaaaaaaaggccaacgc

SEQ ID NO: 116 - DNA, 40 bp, synthetic construct
  source 1..40: mol_type = other DNA
aatgcagacgacaataaacaacaaaaaaaaatgttcagct

SEQ ID NO: 117 - DNA, 40 bp, synthetic construct
  source 1..40: mol_type = other DNA
cccccagcgaaaaaaaaattataccaagcgcgatctttga

SEQ ID NO: 118 - DNA, 40 bp, synthetic construct
  source 1..40: mol_type = other DNA
atacattaatagattagagccgtaaaaaaaacaatagata

SEQ ID NO: 119 - DNA, 40 bp, synthetic construct
  source 1..40: mol_type = other DNA
tggagcaaaaaaaaaaacaagagaatcgatgaagagagtc

SEQ ID NO: 120 - DNA, 40 bp, synthetic construct
  source 1..40: mol_type = other DNA
attgacaaaccaccaccagagccaaaaaaaagccgccagc

SEQ ID NO: 121 - DNA, 40 bp, synthetic construct
  source 1..40: mol_type = other DNA
acagaatgatagcagcaccgtaaaaaaaaaatcagtagcg

SEQ ID NO: 122 - DNA, 41 bp, synthetic construct
  source 1..41: mol_type = other DNA
ttaaagtagcataagttgggtaacgcaaaaaaaacagggtt

SEQ ID NO: 123 - DNA, 41 bp, synthetic construct
  source 1..41: mol_type = other DNA
taatcatacattaatcaaaaatcaggaaaaaaaatctttac

SEQ ID NO: 124 - DNA, 42 bp, synthetic construct
  source 1..42: mol_type = other DNA
aaacgtagaataaaggtgaaaaaaaagcaacatataaaagaa

SEQ ID NO: 125 - DNA, 46 bp, synthetic construct
  source 1..46: mol_type = other DNA
tccacaggtcttcggctacagccctcatagtaaaaaaaatagcgta

SEQ ID NO: 126 - DNA, 46 bp, synthetic construct
  source 1..46: mol_type = other DNA
cttaatgaaaaaaaacgccgctacagggcccatcaatcagcgtact

SEQ ID NO: 127 - DNA, 46 bp, synthetic construct
  source 1..46: mol_type = other DNA
tgtgagttcaatgacgggaataaccttgcttaaaaaaaactgtaaa

SEQ ID NO: 128 - DNA, 46 bp, synthetic construct
  source 1..46: mol_type = other DNA
cctgactatcaacaaatattatagtcagaagaaaaaaaacaaagcg

SEQ ID NO: 129 - DNA, 49 bp, synthetic construct
  source 1..49: mol_type = other DNA
attaagacaccgaaaatctccttattacgcaaaaaaaaagtatgttagc

SEQ ID NO: 130 - DNA, 51 bp, synthetic construct
  source 1..51: mol_type = other DNA
ttcccaggcctttagggtcacgacgttgtaaaaaaaaaaaacgacggccag

SEQ ID NO: 131 - DNA, 51 bp, synthetic construct
  source 1..51: mol_type = other DNA
aaagacaaaagaaaaaaaaggcgaaccatccaagtttccaccagggaggtt

SEQ ID NO: 132 - DNA, 51 bp, synthetic construct
  source 1..51: mol_type = other DNA
gattgcaaaagcacctgtcaaaaagattaagaaaaaaaaaggaagcccgaa

SEQ ID NO: 133 - DNA, 51 bp, synthetic construct
  source 1..51: mol_type = other DNA
tcgtcgcatgagttttctattaattaattttaaaaaaaacccttagaatcc

SEQ ID NO: 134 - DNA, 51 bp, synthetic construct
  source 1..51: mol_type = other DNA
acgatctaacaatatttaaagttttgtcgtcaaaaaaaatttccagacgtt

SEQ ID NO: 135 - DNA, 51 bp, synthetic construct
  source 1..51: mol_type = other DNA
gtcacgctgcgcaaaaaaaagtaaccaccacacctgtaataaatcgccgcg

SEQ ID NO: 136 - DNA, 53 bp, synthetic construct
  source 1..53: mol_type = other DNA
atagtaatgaatccctttaaacagttcagaaaaaaaaaaaacgagaatgacca

SEQ ID NO: 137 - DNA, 35 bp, synthetic construct
  source 1..35: mol_type = other DNA
actgtaggagccacgattggcagtgcctattaaga

SEQ ID NO: 138 - DNA, 35 bp, synthetic construct
  source 1..35: mol_type = other DNA
tattagcccgcctcccagaattgatgatggggttt

SEQ ID NO: 139 - DNA, 35 bp, synthetic construct
  source 1..35: mol_type = other DNA
attcagtggaagaaaataccatgcaaaagaagttt

SEQ ID NO: 140 - DNA, 35 bp, synthetic construct
  source 1..35: mol_type = other DNA
agtagtatgcgattattacgagtttaccagacgac

SEQ ID NO: 141 - DNA, 42 bp, synthetic construct
  source 1..42: mol_type = other DNA
aggaacgcgtcggaaggaagatcgcactcaaatcaatggccc

SEQ ID NO: 142 - DNA, 42 bp, synthetic construct
  source 1..42: mol_type = other DNA
aaatctaagttggcaacgttacagaaggcaggtttttacatc

SEQ ID NO: 143 - DNA, 42 bp, synthetic construct
  source 1..42: mol_type = other DNA
tcgcattgggataggtgcatctgccagttcggaactggactc

SEQ ID NO: 144 - DNA, 42 bp, synthetic construct
  source 1..42: mol_type = other DNA
ccgcctgtaaaatactttacaatggcaatatttgcaatacca

SEQ ID NO: 145 - DNA, 42 bp, synthetic construct
  source 1..42: mol_type = other DNA
ggcaaaaaagaacgcctaaagggagccccgtaaccgtcacgt

SEQ ID NO: 146 - DNA, 42 bp, synthetic construct
  source 1..42: mol_type = other DNA
ccccagccagggcgagttttttggggtccggcctcttctccg

SEQ ID NO: 147 - DNA, 49 bp, synthetic construct
  source 1..49: mol_type = other DNA
acgacttaagtgtcctggagtgagtaaaatcatggctttccagccaggg

SEQ ID NO: 148 - DNA, 49 bp, synthetic construct
  source 1..49: mol_type = other DNA
gccagggtggatgtgtaagcaataaatccacaattgagtgagtgattgc

SEQ ID NO: 149 - DNA, 49 bp, synthetic construct
  source 1..49: mol_type = other DNA
tacgagcgtattaatgaagcccttaccatagacggagggtaattgagcg

SEQ ID NO: 150 - DNA, 49 bp, synthetic construct
  source 1..49: mol_type = other DNA
tagataatttttatacgcgagagttacacagccttttgagttaagccca

SEQ ID NO: 151 - DNA, 28 bp, synthetic construct
  source 1..28: mol_type = other DNA
tagcacccattttcccctcagacaaata

SEQ ID NO: 152 - DNA, 35 bp, synthetic construct
  source 1..35: mol_type = other DNA
tggaacaagagcttgacgggggctagggtgtagcg

SEQ ID NO: 153 - DNA, 35 bp, synthetic construct
  source 1..35: mol_type = other DNA
agacttcttttaatgagagtacctttaaatttagt

SEQ ID NO: 154 - DNA, 35 bp, synthetic construct
  source 1..35: mol_type = other DNA
atcaccgtcaccgactcatacaaatatgcataatc

SEQ ID NO: 155 - DNA, 35 bp, synthetic construct
  source 1..35: mol_type = other DNA
acgttaagagcaagcgctgtgggcgcatccgattt

SEQ ID NO: 156 - DNA, 35 bp, synthetic construct
  source 1..35: mol_type = other DNA
cgtggtgggtaccgcgtgccagaggcggaaagaat

SEQ ID NO: 157 - DNA, 35 bp, synthetic construct
  source 1..35: mol_type = other DNA
tcagctcaaacggcgacgacgacagtatgaggtgc

SEQ ID NO: 158 - DNA, 42 bp, synthetic construct
  source 1..42: mol_type = other DNA
cctgatttagaaccgcagaggcgaattacaaaattaacaatt

SEQ ID NO: 159 - DNA, 42 bp, synthetic construct
  source 1..42: mol_type = other DNA
cgtataaattattcaccctcagaaccgcaagcccaatgtacc

SEQ ID NO: 160 - DNA, 42 bp, synthetic construct
  source 1..42: mol_type = other DNA
tcgcgtcaaatgtggctttccggcaccgctgttggcggtgcg

SEQ ID NO: 161 - DNA, 42 bp, synthetic construct
  source 1..42: mol_type = other DNA
aggcacctgtcgaaaacggtgctgacgaattatacagataca

SEQ ID NO: 162 - DNA, 42 bp, synthetic construct
  source 1..42: mol_type = other DNA
tgccaagctttctcacgaatagaatcggagccggagtaaagc

SEQ ID NO: 163 - DNA, 42 bp, synthetic construct
  source 1..42: mol_type = other DNA
tccttatgttgctaagctacacaaacccataggccctgaaca

SEQ ID NO: 164 - DNA, 42 bp, synthetic construct
  source 1..42: mol_type = other DNA
aacaaagaagagtaatcaacgaaaacgaattcatcgggggta

SEQ ID NO: 165 - DNA, 42 bp, synthetic construct
  source 1..42: mol_type = other DNA
tgacctctgtgtgattgcgttaccagtgtttgatgaaagggc

SEQ ID NO: 166 - DNA, 42 bp, synthetic construct
  source 1..42: mol_type = other DNA
gtaataaaagagaacggaataggtgtatctaatatacaggga

SEQ ID NO: 167 - DNA, 42 bp, synthetic construct
  source 1..42: mol_type = other DNA
tcatcgactcccgactttccacataaaacagagagataaccc

SEQ ID NO: 168 - DNA, 56 bp, synthetic construct
  source 1..56: mol_type = other DNA
gaaccagctgaattgtaagcgcgttacccaaaggataagtgcataataaaaaaatg

SEQ ID NO: 169 - DNA, 56 bp, synthetic construct
  source 1..56: mol_type = other DNA
tcattacggcttatattattttaacgtcgagcaagaaacaatagccgaaagaagga

SEQ ID NO: 170 - DNA, 35 bp, synthetic construct
  source 1..35: mol_type = other DNA
tttagctatagaacctgagtacgcataagaataat

SEQ ID NO: 171 - DNA, 35 bp, synthetic construct
  source 1..35: mol_type = other DNA
tacgtggcactaaattgcgggattgagatttttca

SEQ ID NO: 172 - DNA, 35 bp, synthetic construct
  source 1..35: mol_type = other DNA
atcaattgtcacaccagaacagataccgtccaaaa

SEQ ID NO: 173 - DNA, 35 bp, synthetic construct
  source 1..35: mol_type = other DNA
cgtaaagcactaaattgagggggattgaacagaaa

SEQ ID NO: 174 - DNA, 42 bp, synthetic construct
  source 1..42: mol_type = other DNA
atccgcgacaagaaatataaatcaccagattattcattaaag

SEQ ID NO: 175 - DNA, 42 bp, synthetic construct
  source 1..42: mol_type = other DNA
tacaacgaaccaatatgtaatccaatgaacattcaaccgatt

SEQ ID NO: 176 - DNA, 49 bp, synthetic construct
  source 1..49: mol_type = other DNA
catattctaaagaacggattcgcctgatgataaaataacgccagaataa

SEQ ID NO: 177 - DNA, 49 bp, synthetic construct
  source 1..49: mol_type = other DNA
tttgcggataaatgccctcacagtaacatgccagaagttgagaactgaa

SEQ ID NO: 178 - DNA, 56 bp, synthetic construct
  source 1..56: mol_type = other DNA
ccctgagcaagcgggagcgatgaaggaccatcaccccagccaagcgagtgatgaat

SEQ ID NO: 179 - DNA, 56 bp, synthetic construct
  source 1..56: mol_type = other DNA
atgcgcgactacgacgagggtaattctttttaatgtttgtcacaatcaagacggaa

SEQ ID NO: 180 - DNA, 35 bp, synthetic construct
  source 1..35: mol_type = other DNA
gctgaaatataacaagtggttgtgaattgacagtg

SEQ ID NO: 181 - DNA, 35 bp, synthetic construct
  source 1..35: mol_type = other DNA
acatccataaatatctgaattgtcaacctctaatc

SEQ ID NO: 182 - DNA, 49 bp, synthetic construct
  source 1..49: mol_type = other DNA
atataatttagaagtataagctattcaaaacctgtagctcgaattcgta

SEQ ID NO: 183 - DNA, 49 bp, synthetic construct
  source 1..49: mol_type = other DNA
ttatcataaatcctccccggtgctatttacattaaaattgttatccgct

SEQ ID NO: 184 - DNA, 49 bp, synthetic construct
  source 1..49: mol_type = other DNA
accaaaatagcgagacaataaattgcgttgggaacattttttaatcctg

SEQ ID NO: 185 - DNA, 49 bp, synthetic construct
  source 1..49: mol_type = other DNA
cagttgacagcagcgcctgagaatcggtcgaactccggccctgccatct

SEQ ID NO: 186 - DNA, 49 bp, synthetic construct
  source 1..49: mol_type = other DNA
gagcactggtcagtgccggagaattagctaagctatatttacgctcgcc

SEQ ID NO: 187 - DNA, 56 bp, synthetic construct
  source 1..56: mol_type = other DNA
taaagccagacagccgccgacttgctggtgtagcagcggatggcttagacattcca

SEQ ID NO: 188 - DNA, 56 bp, synthetic construct
  source 1..56: mol_type = other DNA
gcctgttgaggactctttcgaacaggaagccaccgtcaacatgtaaacagagcttt

SEQ ID NO: 189 - DNA, 56 bp, synthetic construct
  source 1..56: mol_type = other DNA
aacatttaattacactatcataaatcgctaccatatggtgtatattttgtaaatca

SEQ ID NO: 190 - DNA, 7560 bp, synthetic construct
  source 1..7560: mol_type = other DNA
agcttggcactggccgtcgttttacaacgtcgtgactgggaaaaccctggcgttacccaacttaatcgccttgcagcacatccccctttcgccagctggcgtaatagcgaagaggcccgcaccgatcgcccttcccaacagttgcgcagcctgaatggcgaatggcgctttgcctggtttccggcaccagaagcggtgccggaaagctggctggagtgcgatcttcctgaggccgatactgtcgtcgtcccctcaaactggcagatgcacggttacgatgcgcccatctacaccaacgtgacctatcccattacggtcaatccgccgtttgttcccacggagaatccgacgggttgttactcgctcacatttaatgttgatgaaagctggctacaggaaggccagacgcgaattatttttgatggcgttcctattggttaaaaaatgagctgatttaacaaaaatttaatgcgaattttaacaaaatattaacgtttacaatttaaatatttgcttatacaatcttcctgtttttggggcttttctgattatcaaccggggtacatatgattgacatgctagttttacgattaccgttcatcgattctcttgtttgctccagactctcaggcaatgacctgatagcctttgtagatctctcaaaaatagctaccctctccggcattaatttatcagctagaacggttgaatatcatattgatggtgatttgactgtctccggcctttctcacccttttgaatctttacctacacattactcaggcattgcatttaaaatatatgagggttctaaaaatttttatccttgcgttgaaataaaggcttctcccgcaaaagtattacagggtcataatgtttttggtacaaccgatttagctttatgctctgaggctttattgcttaattttgctaattctttgccttgcctgtatgatttattggatgttaatgctactactattagtagaattgatgccaccttttcagctcgcgccccaaatgaaaatatagctaaacaggttattgaccatttgcgaaatgtatctaatggtcaaactaaatctactcgttcgcagaattgggaatcaactgttatatggaatgaaacttccagacaccgtactttagttgcatatttaaaacatgttgagctacagcattatattcagcaattaagctctaagccatccgcaaaaatgacctcttatcaaaaggagcaattaaaggtactctctaatcctgacctgttggagtttgcttccggtctggttcgctttgaagctcgaattaaaacgcgatatttgaagtctttcgggcttcctcttaatctttttgatgcaatccgctttgcttctgactataatagtcagggtaaagacctgatttttgatttatggtcattctcgttttctgaactgtttaaagcatttgagggggattcaatgaatatttatgacgattccgcagtattggacgctatccagtctaaacattttactattaccccctctggcaaaacttcttttgcaaaagcctctcgctattttggtttttatcgtcgtctggtaaacgagggttatgatagtgttgctcttactatgcctcgtaattccttttggcgttatgtatctgcattagttgaatgtggtattcctaaatctcaactgatgaatctttctacctgtaataatgttgttccgttagttcgttttattaacgtagatttttcttcccaacgtcctgactggtataatgagccagttcttaaaatcgcataaggtaattcacaatgattaaagttgaaattaaaccatctcaagcccaatttactactcgttctggtgtttctcgtcagggcaagccttattcactgaatgagcagctttgttacgttgatttgggtaatgaatatccggttcttgtcaagattactcttgatgaaggtcagccagcctatgcgcctggtctgtacaccgttcatctgtcctctttcaaagttggtcagttcggttcccttatgattgaccgtctgcgcctcgttccggctaagtaacatggagcaggtcgcggatttcgacacaatttatcaggcgatgatacaaatctccgttgtactttgtttcgcgcttggtataatcgctgggggtcaaagatgagtgttttagtgtattcttttgcctctttcgttttaggttggtgccttcgtagtggcattacgtattttacccgtttaatggaaacttcctcatgaaaaagtctttagtcctcaaagcctctgtagccgttgctaccctcgttccgatgctgtctttcgctgctgagggtgacgatcccgcaaaagcggcctttaactccctgcaagcctcagcgaccgaatatatcggttatgcgtgggcgatggttgttgtcattgtcggcgcaactatcggtatcaagctgtttaagaaattcacctcgaaagcaagctgataaaccgatacaattaaaggctccttttggagccttttttttggagattttcaacgtgaaaaaattattattcgcaattcctttagttgttcctttctattctcactccgctgaaactgttgaaagttgtttagcaaaatcccatacagaaaattcatttactaacgtctggaaagacgacaaaactttagatcgttacgctaactatgagggctgtctgtggaatgctacaggcgttgtagtttgtactggtgacgaaactcagtgttacggtacatgggttcctattgggcttgctatccctgaaaatgagggtggtggctctgagggtggcggttctgagggtggcggttctgagggtggcggtactaaacctcctgagtacggtgatacacctattccgggctatacttatatcaaccctctcgacggcacttatccgcctggtactgagcaaaaccccgctaatcctaatccttctcttgaggagtctcagcctcttaatactttcatgtttcagaataataggttccgaaataggcagggggcattaactgtttatacgggcactgttactcaaggcactgaccccgttaaaacttattaccagtacactcctgtatcatcaaaagccatgtatgacgcttactggaacggtaaattcagagactgcgctttccattctggctttaatgaggatttatttgtttgtgaatatcaaggccaatcgtctgacctgcctcaacctcctgtcaatgctggcggcggctctggtggtggttctggtggcggctctgagggtggtggctctgagggtggcggttctgagggtggcggctctgagggaggcggttccggtggtggctctggttccggtgattttgattatgaaaagatggcaaacgctaataagggggctatgaccgaaaatgccgatgaaaacgcgctacagtctgacgctaaaggcaaacttgattctgtcgctactgattacggtgctgctatcgatggtttcattggtgacgtttccggccttgctaatggtaatggtgctactggtgattttgctggctctaattcccaaatggctcaagtcggtgacggtgataattcacctttaatgaataatttccgtcaatatttaccttccctccctcaatcggttgaatgtcgcccttttgtctttggcgctggtaaaccatatgaattttctattgattgtgacaaaataaacttattccgtggtgtctttgcgtttcttttatatgttgccacctttatgtatgtattttctacgtttgctaacatactgcgtaataaggagtcttaatcatgccagttcttttgggtattccgttattattgcgtttcctcggtttccttctggtaactttgttcggctatctgcttacttttcttaaaaagggcttcggtaagatagctattgctatttcattgtttcttgctcttattattgggcttaactcaattcttgtgggttatctctctgatattagcgctcaattaccctctgactttgttcagggtgttcagttaattctcccgtctaatgcgcttccctgtttttatgttattctctctgtaaaggctgctattttcatttttgacgttaaacaaaaaatcgtttcttatttggattgggataaataatatggctgtttattttgtaactggcaaattaggctctggaaagacgctcgttagcgttggtaagattcaggataaaattgtagctgggtgcaaaatagcaactaatcttgatttaaggcttcaaaacctcccgcaagtcgggaggttcgctaaaacgcctcgcgttcttagaataccggataagccttctatatctgatttgcttgctattgggcgcggtaatgattcctacgatgaaaataaaaacggcttgcttgttctcgatgagtgcggtacttggtttaatacccgttcttggaatgataaggaaagacagccgattattgattggtttctacatgctcgtaaattaggatgggatattatttttcttgttcaggacttatctattgttgataaacaggcgcgttctgcattagctgaacatgttgtttattgtcgtcgtctggacagaattactttaccttttgtcggtactttatattctcttattactggctcgaaaatgcctctgcctaaattacatgttggcgttgttaaatatggcgattctcaattaagccctactgttgagcgttggctttatactggtaagaatttgtataacgcatatgatactaaacaggctttttctagtaattatgattccggtgtttattcttatttaacgccttatttatcacacggtcggtatttcaaaccattaaatttaggtcagaagatgaaattaactaaaatatatttgaaaaagttttctcgcgttctttgtcttgcgattggatttgcatcagcatttacatatagttatataacccaacctaagccggaggttaaaaaggtagtctctcagacctatgattttgataaattcactattgactcttctcagcgtcttaatctaagctatcgctatgttttcaaggattctaagggaaaattaattaatagcgacgatttacagaagcaaggttattcactcacatatattgatttatgtactgtttccattaaaaaaggtaattcaaatgaaattgttaaatgtaattaattttgttttcttgatgtttgtttcatcatcttcttttgctcaggtaattgaaatgaataattcgcctctgcgcgattttgtaacttggtattcaaagcaatcaggcgaatccgttattgtttctcccgatgtaaaaggtactgttactgtatattcatctgacgttaaacctgaaaatctacgcaatttctttatttctgttttacgtgcaaataattttgatatggtaggttctaacccttccattattcagaagtataatccaaacaatcaggattatattgatgaattgccatcatctgataatcaggaatatgatgataattccgctccttctggtggtttctttgttccgcaaaatgataatgttactcaaacttttaaaattaataacgttcgggcaaaggatttaatacgagttgtcgaattgtttgtaaagtctaatacttctaaatcctcaaatgtattatctattgacggctctaatctattagttgttagtgctcctaaagatattttagataaccttcctcaattcctttcaactgttgatttgccaactgaccagatattgattgagggtttgatatttgaggttcagcaaggtgatgctttagatttttcatttgctgctggctctcagcgtggcactgttgcaggcggtgttaatactgaccgcctcacctctgttttatcttctgctggtggttcgttcggtatttttaatggcgatgttttagggctatcagttcgcgcattaaagactaatagccattcaaaaatattgtctgtgccacgtattcttacgctttcaggtcagaagggttctatctctgttggccagaatgtcccttttattactggtcgtgtgactggtgaatctgccaatgtaaataatccatttcagacgattgagcgtcaaaatgtaggtatttccatgagcgtttttcctgttgcaatggctggcggtaatattgttctggatattaccagcaaggccgatagtttgagttcttctactcaggcaagtgatgttattactaatcaaagaagtattgctacaacggttaatttgcgtgatggacagactcttttactcggtggcctcactgattataaaaacacttctcaggattctggcgtaccgttcctgtctaaaatccctttaatcggcctcctgtttagctcccgctctgattctaacgaggaaagcacgttatacgtgctcgtcaaagcaaccatagtacgcgccctgtagcggcgcattaagcgcggcgggtgtggtggttacgcgcagcgtgaccgctacacttgccagcgccctagcgcccgctcctttcgctttcttcccttcctttctcgccacgttcgccggctttccccgtcaagctctaaatcgggggctccctttagggttccgatttagtgctttacggcacctcgaccccaaaaaacttgatttgggtgatggttcacgtagtgggccatcgccctgatagacggtttttcgccctttgacgttggagtccacgttctttaatagtggactcttgttccaaactggaacaacactcaaccctatctcgggctattcttttgatttataagggattttgccgatttcggaaccaccatcaaacaggattttcgcctgctggggcaaaccagcgtggaccgcttgctgcaactctctcagggccaggcggtgaagggcaatcagctgttgcccgtctcactggtgaaaagaaaaaccaccctggcgcccaatacgcaaaccgcctctccccgcgcgttggccgattcattaatgcagctggcacgacaggtttcccgactggaaagcgggcagtgagcgcaacgcaattaatgtgagttagctcactcattaggcaccccaggctttacactttatgcttccggctcgtatgttgtgtggaattgtgagcggataacaatttcacacaggaaacagctatgaccatgattacgaattcgagctcggtacccggggatcctccgtctttatcgaggtaacaagcaccacgtagcttaagccctgtttactcattacaccaaccaggaggtcagagttcggagaaatgatttatgtgaaatgcgtcagccgattcaaggcccctatattcgtgcccaccgacgagttgcttacagatggcagggccgcactgtcggtatcatagagtcactccagggcgagcgtaaatagattagaagcggggttattttggcgggacattgtcataaggttgacaattcagcactaaggacacttaagtcgtgcgcatgaattcacaaccacttagaagaacatccaccctggcttctcctgagaa

SEQ ID NO: 191 - DNA, 64 bp, Homo sapiens
  source 1..64: mol_type = other DNA
tattcataatgtttagactggatagcgtccaataaaagatagcacagcctggatagcaacgtac

SEQ ID NO: 192 - DNA, 64 bp, Homo sapiens
  source 1..64: mol_type = other DNA
aggattatcgagcttcaaagcgaaccagaccggaaaagatagcacagcctggatagcaacgtac

SEQ ID NO: 193 - DNA, 64 bp, Homo sapiens
  source 1..64: mol_type = other DNA
tgcgcaacttctggtgccggaaaccaggcaaagaaaagatagcacagcctggatagcaacgtac

SEQ ID NO: 194 - DNA, 64 bp, Homo sapiens
  source 1..64: mol_type = other DNA
aggaacattttgctaaacaactttcaacagtttaaaagatagcacagcctggatagcaacgtac

SEQ ID NO: 195 - DNA, 64 bp, Homo sapiens
  source 1..64: mol_type = other DNA
ggatagccaccctcagaaccgccaccctcagagaaaagatagcacagcctggatagcaacgtac

SEQ ID NO: 196 - DNA, 64 bp, Homo sapiens
  source 1..64: mol_type = other DNA
aagaaaattcatttcaattacctgagcaaaagaaaaagatagcacagcctggatagcaacgtac

SEQ ID NO: 197 - DNA, 64 bp, Homo sapiens
  source 1..64: mol_type = other DNA
agcagatgaaatagcaatagctatcttaccgaaaaaagatagcacagcctggatagcaacgtac

SEQ ID NO: 198 - DNA, 64 bp, Homo sapiens
  source 1..64: mol_type = other DNA
gtctgagttaagacgctgagaagagtcaatagtaaaagatagcacagcctggatagcaacgtac

SEQ ID NO: 199 - DNA, 64 bp, Homo sapiens
  source 1..64: mol_type = other DNA
agcgggcaaagccggcgaacgtggcgagaaaggaaaagatagcacagcctggatagcaacgtac

SEQ ID NO: 200 - DNA, 64 bp, Homo sapiens
  source 1..64: mol_type = other DNA
agtgtttgattaaagggattttagacaggaacgaaaagatagcacagcctggatagcaacgtac

SEQ ID NO: 201 - DNA, 67 bp, Homo sapiens
  source 1..67: mol_type = other DNA
tattcataatgtttagactggatagcgtccaataaaacaccttctacaatgagctgcgtgtggctcc

SEQ ID NO: 202 - DNA, 67 bp, Homo sapiens
  source 1..67: mol_type = other DNA
aggattatcgagcttcaaagcgaaccagaccggaaaacaccttctacaatgagctgcgtgtggctcc

SEQ ID NO: 203 - DNA, 67 bp, Homo sapiens
  source 1..67: mol_type = other DNA
tgcgcaacttctggtgccggaaaccaggcaaagaaaacaccttctacaatgagctgcgtgtggctcc

SEQ ID NO: 204 - DNA, 67 bp, Homo sapiens
  source 1..67: mol_type = other DNA
aggaacattttgctaaacaactttcaacagtttaaaacaccttctacaatgagctgcgtgtggctcc

SEQ ID NO: 205 - DNA, 67 bp, Homo sapiens
  source 1..67: mol_type = other DNA
ggatagccaccctcagaaccgccaccctcagagaaaacaccttctacaatgagctgcgtgtggctcc

SEQ ID NO: 206 - DNA, 67 bp, Homo sapiens
  source 1..67: mol_type = other DNA
aagaaaattcatttcaattacctgagcaaaagaaaaacaccttctacaatgagctgcgtgtggctcc

SEQ ID NO: 207 - DNA, 67 bp, Homo sapiens
  source 1..67: mol_type = other DNA
agcagatgaaatagcaatagctatcttaccgaaaaaacaccttctacaatgagctgcgtgtggctcc

SEQ ID NO: 208 - DNA, 67 bp, Homo sapiens
  source 1..67: mol_type = other DNA
gtctgagttaagacgctgagaagagtcaatagtaaaacaccttctacaatgagctgcgtgtggctcc

SEQ ID NO: 209 - DNA, 67 bp, Homo sapiens
  source 1..67: mol_type = other DNA
agcgggcaaagccggcgaacgtggcgagaaaggaaaacaccttctacaatgagctgcgtgtggctcc

SEQ ID NO: 210 - DNA, 67 bp, Homo sapiens
  source 1..67: mol_type = other DNA
agtgtttgattaaagggattttagacaggaacgaaaacaccttctacaatgagctgcgtgtggctcc

SEQ ID NO: 211 - DNA, 67 bp, Homo sapiens
  source 1..67: mol_type = other DNA
tattcataatgtttagactggatagcgtccaataaaattaatgtcacgcacgatttcccgctcggcc

SEQ ID NO: 212 - DNA, 67 bp, Homo sapiens
  source 1..67: mol_type = other DNA
aggattatcgagcttcaaagcgaaccagaccggaaaattaatgtcacgcacgatttcccgctcggcc

SEQ ID NO: 213 - DNA, 67 bp, Homo sapiens
  source 1..67: mol_type = other DNA
tgcgcaacttctggtgccggaaaccaggcaaagaaaattaatgtcacgcacgatttcccgctcggcc

SEQ ID NO: 214 - DNA, 67 bp, Homo sapiens
  source 1..67: mol_type = other DNA
aggaacattttgctaaacaactttcaacagtttaaaattaatgtcacgcacgatttcccgctcggcc

SEQ ID NO: 215 - DNA, 67 bp, Homo sapiens
  source 1..67: mol_type = other DNA
ggatagccaccctcagaaccgccaccctcagagaaaattaatgtcacgcacgatttcccgctcggcc

SEQ ID NO: 216 - DNA, 67 bp, Homo sapiens
  source 1..67: mol_type = other DNA
aagaaaattcatttcaattacctgagcaaaagaaaaattaatgtcacgcacgatttcccgctcggcc

SEQ ID NO: 217 - DNA, 67 bp, Homo sapiens
  source 1..67: mol_type = other DNA
agcagatgaaatagcaatagctatcttaccgaaaaaattaatgtcacgcacgatttcccgctcggcc

SEQ ID NO: 218 - DNA, 67 bp, Homo sapiens
  source 1..67: mol_type = other DNA
gtctgagttaagacgctgagaagagtcaatagtaaaattaatgtcacgcacgatttcccgctcggcc

SEQ ID NO: 219 - DNA, 67 bp, Homo sapiens
  source 1..67: mol_type = other DNA
agcgggcaaagccggcgaacgtggcgagaaaggaaaattaatgtcacgcacgatttcccgctcggcc

SEQ ID NO: 220 - DNA, 67 bp, Homo sapiens
  source 1..67: mol_type = other DNA
agtgtttgattaaagggattttagacaggaacgaaaattaatgtcacgcacgatttcccgctcggcc

SEQ ID NO: 221 - DNA, 67 bp, Homo sapiens
  source 1..67: mol_type = other DNA
tattcataatgtttagactggatagcgtccaataaaagtggtaactcggacattgattggtttcggc

SEQ ID NO: 222 - DNA, 67 bp, Homo sapiens
  source 1..67: mol_type = other DNA
aggattatcgagcttcaaagcgaaccagaccggaaaagtggtaactcggacattgattggtttcggc

SEQ ID NO: 223 - DNA, 67 bp, Homo sapiens
  source 1..67: mol_type = other DNA
tgcgcaacttctggtgccggaaaccaggcaaagaaaagtggtaactcggacattgattggtttcggc

SEQ ID NO: 224 - DNA, 67 bp, Homo sapiens
  source 1..67: mol_type = other DNA
aggaacattttgctaaacaactttcaacagtttaaaagtggtaactcggacattgattggtttcggc

SEQ ID NO: 225 - DNA, 67 bp, Homo sapiens
  source 1..67: mol_type = other DNA
ggatagccaccctcagaaccgccaccctcagagaaaagtggtaactcggacattgattggtttcggc

SEQ ID NO: 226 - DNA, 67 bp, Homo sapiens
  source 1..67: mol_type = other DNA
aagaaaattcatttcaattacctgagcaaaagaaaaagtggtaactcggacattgattggtttcggc

SEQ ID NO: 227 - DNA, 67 bp, Homo sapiens
  source 1..67: mol_type = other DNA
agcagatgaaatagcaatagctatcttaccgaaaaaagtggtaactcggacattgattggtttcggc

SEQ ID NO: 228 - DNA, 67 bp, Homo sapiens
  source 1..67: mol_type = other DNA
gtctgagttaagacgctgagaagagtcaatagtaaaagtggtaactcggacattgattggtttcggc

SEQ ID NO: 229 - DNA, 67 bp, Homo sapiens
  source 1..67: mol_type = other DNA
agcgggcaaagccggcgaacgtggcgagaaaggaaaagtggtaactcggacattgattggtttcggc

SEQ ID NO: 230 - DNA, 67 bp, Homo sapiens
  source 1..67: mol_type = other DNA
agtgtttgattaaagggattttagacaggaacgaaaagtggtaactcggacattgattggtttcggc

SEQ ID NO: 231 - DNA, 67 bp, Homo sapiens
  source 1..67: mol_type = other DNA
tattcataatgtttagactggatagcgtccaataaaaccagttgtatttggctggattgcaaactcc

SEQ ID NO: 232 - DNA, 67 bp, Homo sapiens
  source 1..67: mol_type = other DNA
aggattatcgagcttcaaagcgaaccagaccggaaaaccagttgtatttggctggattgcaaactcc

SEQ ID NO: 233 - DNA, 67 bp, Homo sapiens
  source 1..67: mol_type = other DNA
tgcgcaacttctggtgccggaaaccaggcaaagaaaaccagttgtatttggctggattgcaaactcc

SEQ ID NO: 234 - DNA, 67 bp, Homo sapiens
  source 1..67: mol_type = other DNA
aggaacattttgctaaacaactttcaacagtttaaaaccagttgtatttggctggattgcaaactcc

SEQ ID NO: 235 - DNA, 67 bp, Homo sapiens
  source 1..67: mol_type = other DNA
ggatagccaccctcagaaccgccaccctcagagaaaaccagttgtatttggctggattgcaaactcc

SEQ ID NO: 236 - DNA, 67 bp, Homo sapiens
  source 1..67: mol_type = other DNA
aagaaaattcatttcaattacctgagcaaaagaaaaaccagttgtatttggctggattgcaaactcc

SEQ ID NO: 237 - DNA, 67 bp, Homo sapiens
  source 1..67: mol_type = other DNA
agcagatgaaatagcaatagctatcttaccgaaaaaaccagttgtatttggctggattgcaaactcc

SEQ ID NO: 238 - DNA, 67 bp, Homo sapiens
  source 1..67: mol_type = other DNA
gtctgagttaagacgctgagaagagtcaatagtaaaaccagttgtatttggctggattgcaaactcc

SEQ ID NO: 239 - DNA, 67 bp, Homo sapiens
  source 1..67: mol_type = other DNA
agcgggcaaagccggcgaacgtggcgagaaaggaaaaccagttgtatttggctggattgcaaactcc

SEQ ID NO: 240 - DNA, 67 bp, Homo sapiens
  source 1..67: mol_type = other DNA
agtgtttgattaaagggattttagacaggaacgaaaaccagttgtatttggctggattgcaaactcc

SEQ ID NO: 241 - DNA, 67 bp, Homo sapiens
  source 1..67: mol_type = other DNA
tattcataatgtttagactggatagcgtccaataaaactgcggcgcatatacaactcatggttgccc

SEQ ID NO: 242 - DNA, 67 bp, Homo sapiens
  source 1..67: mol_type = other DNA
aggattatcgagcttcaaagcgaaccagaccggaaaactgcggcgcatatacaactcatggttgccc

SEQ ID NO: 243 - DNA, 67 bp, Homo sapiens
  source 1..67: mol_type = other DNA
tgcgcaacttctggtgccggaaaccaggcaaagaaaactgcggcgcatatacaactcatggttgccc

SEQ ID NO: 244 - DNA, 67 bp, Homo sapiens
  source 1..67: mol_type = other DNA
aggaacattttgctaaacaactttcaacagtttaaaactgcggcgcatatacaactcatggttgccc

SEQ ID NO: 245 - DNA, 67 bp, Homo sapiens
  source 1..67: mol_type = other DNA
ggatagccaccctcagaaccgccaccctcagagaaaactgcggcgcatatacaactcatggttgccc

SEQ ID NO: 246 - DNA, 67 bp, Homo sapiens
  source 1..67: mol_type = other DNA
aagaaaattcatttcaattacctgagcaaaagaaaaactgcggcgcatatacaactcatggttgccc

SEQ ID NO: 247 - DNA, 67 bp, Homo sapiens
  source 1..67: mol_type = other DNA
agcagatgaaatagcaatagctatcttaccgaaaaaactgcggcgcatatacaactcatggttgccc

SEQ ID NO: 248 - DNA, 67 bp, Homo sapiens
  source 1..67: mol_type = other DNA
gtctgagttaagacgctgagaagagtcaatagtaaaactgcggcgcatatacaactcatggttgccc

SEQ ID NO: 249 - DNA, 67 bp, Homo sapiens
  source 1..67: mol_type = other DNA
agcgggcaaagccggcgaacgtggcgagaaaggaaaactgcggcgcatatacaactcatggttgccc

SEQ ID NO: 250 - DNA, 67 bp, Homo sapiens
  source 1..67: mol_type = other DNA
agtgtttgattaaagggattttagacaggaacgaaaactgcggcgcatatacaactcatggttgccc

SEQ ID NO: 251 - DNA, 67 bp, Homo sapiens
  source 1..67: mol_type = other DNA
tattcataatgtttagactggatagcgtccaataaaaaatattgtgaagcttgtagtagagcccaca

SEQ ID NO: 252 - DNA, 67 bp, Homo sapiens
  source 1..67: mol_type = other DNA
aggattatcgagcttcaaagcgaaccagaccggaaaaaatattgtgaagcttgtagtagagcccaca

SEQ ID NO: 253 - DNA, 67 bp, Homo sapiens
  source 1..67: mol_type = other DNA
tgcgcaacttctggtgccggaaaccaggcaaagaaaaaatattgtgaagcttgtagtagagcccaca

SEQ ID NO: 254 - DNA, 67 bp, Homo sapiens
  source 1..67: mol_type = other DNA
aggaacattttgctaaacaactttcaacagtttaaaaaatattgtgaagcttgtagtagagcccaca

SEQ ID NO: 255 - DNA, 67 bp, Homo sapiens
  source 1..67: mol_type = other DNA
ggatagccaccctcagaaccgccaccctcagagaaaaaatattgtgaagcttgtagtagagcccaca

SEQ ID NO: 256 - DNA, 67 bp, Homo sapiens
  source 1..67: mol_type = other DNA
aagaaaattcatttcaattacctgagcaaaagaaaaaaatattgtgaagcttgtagtagagcccaca

SEQ ID NO: 257 - DNA, 67 bp, Homo sapiens
  source 1..67: mol_type = other DNA
agcagatgaaatagcaatagctatcttaccgaaaaaaaatattgtgaagcttgtagtagagcccaca

SEQ ID NO: 258 - DNA, 67 bp, Homo sapiens
  source 1..67: mol_type = other DNA
gtctgagttaagacgctgagaagagtcaatagtaaaaaatattgtgaagcttgtagtagagcccaca

SEQ ID NO: 259 - DNA, 67 bp, Homo sapiens
  source 1..67: mol_type = other DNA
agcgggcaaagccggcgaacgtggcgagaaaggaaaaaatattgtgaagcttgtagtagagcccaca

SEQ ID NO: 260 - DNA, 67 bp, Homo sapiens
  source 1..67: mol_type = other DNA
agtgtttgattaaagggattttagacaggaacgaaaaaatattgtgaagcttgtagtagagcccaca

SEQ ID NO: 261 - DNA, 67 bp, Homo sapiens
  source 1..67: mol_type = other DNA
tattcataatgtttagactggatagcgtccaataaaatggatttgctagacatttttcggtttctgg

SEQ ID NO: 262 - DNA, 67 bp, Homo sapiens
  source 1..67: mol_type = other DNA
aggattatcgagcttcaaagcgaaccagaccggaaaatggatttgctagacatttttcggtttctgg

SEQ ID NO: 263 - DNA, 67 bp, Homo sapiens
  source 1..67: mol_type = other DNA
tgcgcaacttctggtgccggaaaccaggcaaagaaaatggatttgctagacatttttcggtttctgg

SEQ ID NO: 264 - DNA, 67 bp, Homo sapiens
  source 1..67: mol_type = other DNA
aggaacattttgctaaacaactttcaacagtttaaaatggatttgctagacatttttcggtttctgg

SEQ ID NO: 265 - DNA, 67 bp, Homo sapiens
  source 1..67: mol_type = other DNA
ggatagccaccctcagaaccgccaccctcagagaaaatggatttgctagacatttttcggtttctgg

SEQ ID NO: 266 - DNA, 67 bp, Homo sapiens
  source 1..67: mol_type = other DNA
aagaaaattcatttcaattacctgagcaaaagaaaaatggatttgctagacatttttcggtttctgg

SEQ ID NO: 267 - DNA, 67 bp, Homo sapiens
  source 1..67: mol_type = other DNA
agcagatgaaatagcaatagctatcttaccgaaaaaatggatttgctagacatttttcggtttctgg

SEQ ID NO: 268 - DNA, 67 bp, Homo sapiens
  source 1..67: mol_type = other DNA
gtctgagttaagacgctgagaagagtcaatagtaaaatggatttgctagacatttttcggtttctgg

SEQ ID NO: 269 - DNA, 67 bp, Homo sapiens
  source 1..67: mol_type = other DNA
agcgggcaaagccggcgaacgtggcgagaaaggaaaatggatttgctagacatttttcggtttctgg

SEQ ID NO: 270 - DNA, 67 bp, Homo sapiens
  source 1..67: mol_type = other DNA
agtgtttgattaaagggattttagacaggaacgaaaatggatttgctagacatttttcggtttctgg

SEQ ID NO: 271 - DNA, 67 bp, Homo sapiens
  source 1..67: mol_type = other DNA
tattcataatgtttagactggatagcgtccaataaaactcctgtttttatcaatggtgcactggttg

SEQ ID NO: 272 - DNA, 67 bp, Homo sapiens
  source 1..67: mol_type = other DNA
aggattatcgagcttcaaagcgaaccagaccggaaaactcctgtttttatcaatggtgcactggttg

SEQ ID NO: 273 - DNA, 67 bp, Homo sapiens
  source 1..67: mol_type = other DNA
tgcgcaacttctggtgccggaaaccaggcaaagaaaactcctgtttttatcaatggtgcactggttg

SEQ ID NO: 274 - DNA, 67 bp, Homo sapiens
  source 1..67: mol_type = other DNA
aggaacattttgctaaacaactttcaacagtttaaaactcctgtttttatcaatggtgcactggttg

SEQ ID NO: 275 - DNA, 67 bp, Homo sapiens
  source 1..67: mol_type = other DNA
ggatagccaccctcagaaccgccaccctcagagaaaactcctgtttttatcaatggtgcactggttg

SEQ ID NO: 276 - DNA, 67 bp, Homo sapiens
  source 1..67: mol_type = other DNA
aagaaaattcatttcaattacctgagcaaaagaaaaactcctgtttttatcaatggtgcactggttg

SEQ ID NO: 277 - DNA, 67 bp, Homo sapiens
  source 1..67: mol_type = other DNA
agcagatgaaatagcaatagctatcttaccgaaaaaactcctgtttttatcaatggtgcactggttg

SEQ ID NO: 278 - DNA, 67 bp, Homo sapiens
  source 1..67: mol_type = other DNA
gtctgagttaagacgctgagaagagtcaatagtaaaactcctgtttttatcaatggtgcactggttg

SEQ ID NO: 279 - DNA, 67 bp, Homo sapiens
  source 1..67: mol_type = other DNA
agcgggcaaagccggcgaacgtggcgagaaaggaaaactcctgtttttatcaatggtgcactggttg

SEQ ID NO: 280 - DNA, 67 bp, Homo sapiens
  source 1..67: mol_type = other DNA
agtgtttgattaaagggattttagacaggaacgaaaactcctgtttttatcaatggtgcactggttg

SEQ ID NO: 281 - DNA, 67 bp, Homo sapiens
  source 1..67: mol_type = other DNA
tattcataatgtttagactggatagcgtccaataaaacgattatctgaatttggcctgtagaatgcc

SEQ ID NO: 282 - DNA, 67 bp, Homo sapiens
  source 1..67: mol_type = other DNA
aggattatcgagcttcaaagcgaaccagaccggaaaacgattatctgaatttggcctgtagaatgcc

SEQ ID NO: 283 - DNA, 67 bp, Homo sapiens
  source 1..67: mol_type = other DNA
tgcgcaacttctggtgccggaaaccaggcaaagaaaacgattatctgaatttggcctgtagaatgcc

SEQ ID NO: 284 - DNA, 67 bp, Homo sapiens
  source 1..67: mol_type = other DNA
aggaacattttgctaaacaactttcaacagtttaaaacgattatctgaatttggcctgtagaatgcc

SEQ ID NO: 285 - DNA, 67 bp, Homo sapiens
  source 1..67: mol_type = other DNA
ggatagccaccctcagaaccgccaccctcagagaaaacgattatctgaatttggcctgtagaatgcc

SEQ ID NO: 286 - DNA, 67 bp, Homo sapiens
  source 1..67: mol_type = other DNA
aagaaaattcatttcaattacctgagcaaaagaaaaacgattatctgaatttggcctgtagaatgcc

SEQ ID NO: 287 - DNA, 67 bp, Homo sapiens
  source 1..67: mol_type = other DNA
agcagatgaaatagcaatagctatcttaccgaaaaaacgattatctgaatttggcctgtagaatgcc

SEQ ID NO: 288 - DNA, 67 bp, Homo sapiens
  source 1..67: mol_type = other DNA
gtctgagttaagacgctgagaagagtcaatagtaaaacgattatctgaatttggcctgtagaatgcc

SEQ ID NO: 289 - DNA, 67 bp, Homo sapiens
  source 1..67: mol_type = other DNA
agcgggcaaagccggcgaacgtggcgagaaaggaaaacgattatctgaatttggcctgtagaatgcc

SEQ ID NO: 290 - DNA, 67 bp, Homo sapiens
  source 1..67: mol_type = other DNA
agtgtttgattaaagggattttagacaggaacgaaaacgattatctgaatttggcctgtagaatgcc

SEQ ID NO: 291 - DNA, 67 bp, Homo sapiens
  source 1..67: mol_type = other DNA
tattcataatgtttagactggatagcgtccaataaaacttcttgatgtcatcatatttggcaggttt

SEQ ID NO: 292 - DNA, 67 bp, Homo sapiens
  source 1..67: mol_type = other DNA
aggattatcgagcttcaaagcgaaccagaccggaaaacttcttgatgtcatcatatttggcaggttt

SEQ ID NO: 293 - DNA, 67 bp, Homo sapiens
  source 1..67: mol_type = other DNA
tgcgcaacttctggtgccggaaaccaggcaaagaaaacttcttgatgtcatcatatttggcaggttt

SEQ ID NO: 294 - DNA, 67 bp, Homo sapiens
  source 1..67: mol_type = other DNA
aggaacattttgctaaacaactttcaacagtttaaaacttcttgatgtcatcatatttggcaggttt

SEQ ID NO: 295 - DNA, 67 bp, Homo sapiens
  source 1..67: mol_type = other DNA
ggatagccaccctcagaaccgccaccctcagagaaaacttcttgatgtcatcatatttggcaggttt

SEQ ID NO: 296 - DNA, 67 bp, Homo sapiens
  source 1..67: mol_type = other DNA
aagaaaattcatttcaattacctgagcaaaagaaaaacttcttgatgtcatcatatttggcaggttt

SEQ ID NO: 297 - DNA, 67 bp, Homo sapiens
  source 1..67: mol_type = other DNA
agcagatgaaatagcaatagctatcttaccgaaaaaacttcttgatgtcatcatatttggcaggttt

SEQ ID NO: 298 - DNA, 67 bp, Homo sapiens
  source 1..67: mol_type = other DNA
gtctgagttaagacgctgagaagagtcaatagtaaaacttcttgatgtcatcatatttggcaggttt

SEQ ID NO: 299 - DNA, 67 bp, Homo sapiens
  source 1..67: mol_type = other DNA
agcgggcaaagccggcgaacgtggcgagaaaggaaaacttcttgatgtcatcatatttggcaggttt

SEQ ID NO: 300 - DNA, 67 bp, Homo sapiens
  source 1..67: mol_type = other DNA
agtgtttgattaaagggattttagacaggaacgaaaacttcttgatgtcatcatatttggcaggttt

SEQ ID NO: 301 - DNA, 67 bp, Homo sapiens
  source 1..67: mol_type = other DNA
tattcataatgtttagactggatagcgtccaataaaatcgctgttgaagtcagaggagaccacctgg

SEQ ID NO: 302 - DNA, 67 bp, Homo sapiens
  source 1..67: mol_type = other DNA
aggattatcgagcttcaaagcgaaccagaccggaaaatcgctgttgaagtcagaggagaccacctgg

SEQ ID NO: 303 - DNA, 67 bp, Homo sapiens
  source 1..67: mol_type = other DNA
tgcgcaacttctggtgccggaaaccaggcaaagaaaatcgctgttgaagtcagaggagaccacctgg

SEQ ID NO: 304 - DNA, 67 bp, Homo sapiens
  source 1..67: mol_type = other DNA
aggaacattttgctaaacaactttcaacagtttaaaatcgctgttgaagtcagaggagaccacctgg

SEQ ID NO: 305 - DNA, 67 bp, Homo sapiens
  source 1..67: mol_type = other DNA
ggatagccaccctcagaaccgccaccctcagagaaaatcgctgttgaagtcagaggagaccacctgg

SEQ ID NO: 306 - DNA, 67 bp, Homo sapiens
  source 1..67: mol_type = other DNA
aagaaaattcatttcaattacctgagcaaaagaaaaatcgctgttgaagtcagaggagaccacctgg

SEQ ID NO: 307 - DNA, 67 bp, Homo sapiens
  source 1..67: mol_type = other DNA
agcagatgaaatagcaatagctatcttaccgaaaaaatcgctgttgaagtcagaggagaccacctgg

SEQ ID NO: 308 - DNA, 67 bp, Homo sapiens
  source 1..67: mol_type = other DNA
gtctgagttaagacgctgagaagagtcaatagtaaaatcgctgttgaagtcagaggagaccacctgg

SEQ ID NO: 309 - DNA, 67 bp, Homo sapiens
  source 1..67: mol_type = other DNA
agcgggcaaagccggcgaacgtggcgagaaaggaaaatcgctgttgaagtcagaggagaccacctgg

SEQ ID NO: 310 - DNA, 67 bp, Homo sapiens
  source 1..67: mol_type = other DNA
agtgtttgattaaagggattttagacaggaacgaaaatcgctgttgaagtcagaggagaccacctgg

SEQ ID NO: 311 - DNA, 67 bp, Homo sapiens
  source 1..67: mol_type = other DNA
tattcataatgtttagactggatagcgtccaataaaatccaaggcatcaccaagattaaagtcctcg

SEQ ID NO: 312 - DNA, 67 bp, Homo sapiens
  source 1..67: mol_type = other DNA
aggattatcgagcttcaaagcgaaccagaccggaaaatccaaggcatcaccaagattaaagtcctcg

SEQ ID NO: 313 - DNA, 67 bp, Homo sapiens
  source 1..67: mol_type = other DNA
tgcgcaacttctggtgccggaaaccaggcaaagaaaatccaaggcatcaccaagattaaagtcctcg

SEQ ID NO: 314 - DNA, 67 bp, Homo sapiens
  source 1..67: mol_type = other DNA
aggaacattttgctaaacaactttcaacagtttaaaatccaaggcatcaccaagattaaagtcctcg

SEQ ID NO: 315 - DNA, 67 bp, Homo sapiens
  source 1..67: mol_type = other DNA
ggatagccaccctcagaaccgccaccctcagagaaaatccaaggcatcaccaagattaaagtcctcg

SEQ ID NO: 316 - DNA, 67 bp, Homo sapiens
  source 1..67: mol_type = other DNA
aagaaaattcatttcaattacctgagcaaaagaaaaatccaaggcatcaccaagattaaagtcctcg

SEQ ID NO: 317 - DNA, 67 bp, Homo sapiens
  source 1..67: mol_type = other DNA
agcagatgaaatagcaatagctatcttaccgaaaaaatccaaggcatcaccaagattaaagtcctcg

SEQ ID NO: 318 - DNA, 67 bp, Homo sapiens
  source 1..67: mol_type = other DNA
gtctgagttaagacgctgagaagagtcaatagtaaaatccaaggcatcaccaagattaaagtcctcg

SEQ ID NO: 319 - DNA, 67 bp, Homo sapiens
  source 1..67: mol_type = other DNA
agcgggcaaagccggcgaacgtggcgagaaaggaaaatccaaggcatcaccaagattaaagtcctcg

SEQ ID NO: 320 - DNA, 67 bp, Homo sapiens
  source 1..67: mol_type = other DNA
agtgtttgattaaagggattttagacaggaacgaaaatccaaggcatcaccaagattaaagtcctcg

SEQ ID NO: 321 - DNA, 67 bp, Homo sapiens
  source 1..67: mol_type = other DNA
tattcataatgtttagactggatagcgtccaataaaatcgtgtgatattggtgtcatcaatgacctt

SEQ ID NO: 322 - DNA, 67 bp, Homo sapiens
  source 1..67: mol_type = other DNA
aggattatcgagcttcaaagcgaaccagaccggaaaatcgtgtgatattggtgtcatcaatgacctt

SEQ ID NO: 323 - DNA, 67 bp, Homo sapiens
  source 1..67: mol_type = other DNA
tgcgcaacttctggtgccggaaaccaggcaaagaaaatcgtgtgatattggtgtcatcaatgacctt

SEQ ID NO: 324 - DNA, 67 bp, Homo sapiens
  source 1..67: mol_type = other DNA
aggaacattttgctaaacaactttcaacagtttaaaatcgtgtgatattggtgtcatcaatgacctt

SEQ ID NO: 325 - DNA, 67 bp, Homo sapiens
  source 1..67: mol_type = other DNA
ggatagccaccctcagaaccgccaccctcagagaaaatcgtgtgatattggtgtcatcaatgacctt

SEQ ID NO: 326 - DNA, 67 bp, Homo sapiens
  source 1..67: mol_type = other DNA
aagaaaattcatttcaattacctgagcaaaagaaaaatcgtgtgatattggtgtcatcaatgacctt

SEQ ID NO: 327 - DNA, 67 bp, Homo sapiens
  source 1..67: mol_type = other DNA
agcagatgaaatagcaatagctatcttaccgaaaaaatcgtgtgatattggtgtcatcaatgacctt

SEQ ID NO: 328 - DNA, 67 bp, Homo sapiens
  source 1..67: mol_type = other DNA
gtctgagttaagacgctgagaagagtcaatagtaaaatcgtgtgatattggtgtcatcaatgacctt

SEQ ID NO: 329 - DNA, 67 bp, Homo sapiens
  source 1..67: mol_type = other DNA
agcgggcaaagccggcgaacgtggcgagaaaggaaaatcgtgtgatattggtgtcatcaatgacctt

SEQ ID NO: 330 - DNA, 67 bp, Homo sapiens
  source 1..67: mol_type = other DNA
agtgtttgattaaagggattttagacaggaacgaaaatcgtgtgatattggtgtcatcaatgacctt

SEQ ID NO: 331 - DNA, 67 bp, Homo sapiens
  source 1..67: mol_type = other DNA
tattcataatgtttagactggatagcgtccaataaaacagacaaattgttgtagtgatcttcctgtc

SEQ ID NO: 332 - DNA, 67 bp, Homo sapiens
  source 1..67: mol_type = other DNA
aggattatcgagcttcaaagcgaaccagaccggaaaacagacaaattgttgtagtgatcttcctgtc

SEQ ID NO: 333 - DNA, 67 bp, Homo sapiens
  source 1..67: mol_type = other DNA
tgcgcaacttctggtgccggaaaccaggcaaagaaaacagacaaattgttgtagtgatcttcctgtc

SEQ ID NO: 334 - DNA, 67 bp, Homo sapiens
  source 1..67: mol_type = other DNA
aggaacattttgctaaacaactttcaacagtttaaaacagacaaattgttgtagtgatcttcctgtc

SEQ ID NO: 335 - DNA, 67 bp, Homo sapiens
  source 1..67: mol_type = other DNA
ggatagccaccctcagaaccgccaccctcagagaaaacagacaaattgttgtagtgatcttcctgtc

SEQ ID NO: 336 - DNA, 67 bp, Homo sapiens
  source 1..67: mol_type = other DNA
aagaaaattcatttcaattacctgagcaaaagaaaaacagacaaattgttgtagtgatcttcctgtc

SEQ ID NO: 337 - DNA, 67 bp, Homo sapiens
  source 1..67: mol_type = other DNA
agcagatgaaatagcaatagctatcttaccgaaaaaacagacaaattgttgtagtgatcttcctgtc

SEQ ID NO: 338 - DNA, 67 bp, Homo sapiens
  source 1..67: mol_type = other DNA
gtctgagttaagacgctgagaagagtcaatagtaaaacagacaaattgttgtagtgatcttcctgtc

SEQ ID NO: 339 - DNA, 67 bp, Homo sapiens
  source 1..67: mol_type = other DNA
agcgggcaaagccggcgaacgtggcgagaaaggaaaacagacaaattgttgtagtgatcttcctgtc

SEQ ID NO: 340 - DNA, 67 bp, Homo sapiens
  source 1..67: mol_type = other DNA
agtgtttgattaaagggattttagacaggaacgaaaacagacaaattgttgtagtgatcttcctgtc

SEQ ID NO: 341 - DNA, 67 bp, Homo sapiens
  source 1..67: mol_type = other DNA
tattcataatgtttagactggatagcgtccaataaaatctcaatggtggcaccaagaatcttgtccc

SEQ ID NO: 342 - DNA, 67 bp, Homo sapiens
  source 1..67: mol_type = other DNA
aggattatcgagcttcaaagcgaaccagaccggaaaatctcaatggtggcaccaagaatcttgtccc

SEQ ID NO: 343 - DNA, 67 bp, Homo sapiens
  source 1..67: mol_type = other DNA
tgcgcaacttctggtgccggaaaccaggcaaagaaaatctcaatggtggcaccaagaatcttgtccc

SEQ ID NO: 344 - DNA, 67 bp, Homo sapiens
  source 1..67: mol_type = other DNA
aggaacattttgctaaacaactttcaacagtttaaaatctcaatggtggcaccaagaatcttgtccc

SEQ ID NO: 345 - DNA, 67 bp, Homo sapiens
  source 1..67: mol_type = other DNA
ggatagccaccctcagaaccgccaccctcagagaaaatctcaatggtggcaccaagaatcttgtccc

SEQ ID NO: 346 - DNA, 67 bp, Homo sapiens
  source 1..67: mol_type = other DNA
aagaaaattcatttcaattacctgagcaaaagaaaaatctcaatggtggcaccaagaatcttgtccc

SEQ ID NO: 347 - DNA, 67 bp, Homo sapiens
  source 1..67: mol_type = other DNA
agcagatgaaatagcaatagctatcttaccgaaaaaatctcaatggtggcaccaagaatcttgtccc

SEQ ID NO: 348 - DNA, 67 bp, Homo sapiens
  source 1..67: mol_type = other DNA
gtctgagttaagacgctgagaagagtcaatagtaaaatctcaatggtggcaccaagaatcttgtccc

SEQ ID NO: 349 - DNA, 67 bp, Homo sapiens
  source 1..67: mol_type = other DNA
agcgggcaaagccggcgaacgtggcgagaaaggaaaatctcaatggtggcaccaagaatcttgtccc

SEQ ID NO: 350 - DNA, 67 bp, Homo sapiens
  source 1..67: mol_type = other DNA
agtgtttgattaaagggattttagacaggaacgaaaatctcaatggtggcaccaagaatcttgtccc

SEQ ID NO: 351 - DNA, 67 bp, Homo sapiens
  source 1..67: mol_type = other DNA
tattcataatgtttagactggatagcgtccaataaaaaggtaatgactcgaagctgtattgtgggct

SEQ ID NO: 352 - DNA, 67 bp, Homo sapiens
  source 1..67: mol_type = other DNA
aggattatcgagcttcaaagcgaaccagaccggaaaaaggtaatgactcgaagctgtattgtgggct

SEQ ID NO: 353 - DNA, 67 bp, Homo sapiens
  source 1..67: mol_type = other DNA
tgcgcaacttctggtgccggaaaccaggcaaagaaaaaggtaatgactcgaagctgtattgtgggct

SEQ ID NO: 354 - DNA, 67 bp, Homo sapiens
  source 1..67: mol_type = other DNA
aggaacattttgctaaacaactttcaacagtttaaaaaggtaatgactcgaagctgtattgtgggct

SEQ ID NO: 355 - DNA, 67 bp, Homo sapiens
  source 1..67: mol_type = other DNA
ggatagccaccctcagaaccgccaccctcagagaaaaaggtaatgactcgaagctgtattgtgggct

SEQ ID NO: 356 - DNA, 67 bp, Homo sapiens
  source 1..67: mol_type = other DNA
aagaaaattcatttcaattacctgagcaaaagaaaaaaggtaatgactcgaagctgtattgtgggct

SEQ ID NO: 357 - DNA, 67 bp, Homo sapiens
  source 1..67: mol_type = other DNA
agcagatgaaatagcaatagctatcttaccgaaaaaaaggtaatgactcgaagctgtattgtgggct

SEQ ID NO: 358 - DNA, 67 bp, Homo sapiens
  source 1..67: mol_type = other DNA
gtctgagttaagacgctgagaagagtcaatagtaaaaaggtaatgactcgaagctgtattgtgggct

SEQ ID NO: 359 - DNA, 67 bp, Homo sapiens
  source 1..67: mol_type = other DNA
agcgggcaaagccggcgaacgtggcgagaaaggaaaaaggtaatgactcgaagctgtattgtgggct

SEQ ID NO: 360 - DNA, 67 bp, Homo sapiens
  source 1..67: mol_type = other DNA
agtgtttgattaaagggattttagacaggaacgaaaaaggtaatgactcgaagctgtattgtgggct

SEQ ID NO: 361 - DNA, 67 bp, Homo sapiens
  source 1..67: mol_type = other DNA
tattcataatgtttagactggatagcgtccaataaaaggcaggataggcacgtggatgaaatccatc

SEQ ID NO: 362 - DNA, 67 bp, Homo sapiens
  source 1..67: mol_type = other DNA
aggattatcgagcttcaaagcgaaccagaccggaaaaggcaggataggcacgtggatgaaatccatc

SEQ ID NO: 363 - DNA, 67 bp, Homo sapiens
  source 1..67: mol_type = other DNA
tgcgcaacttctggtgccggaaaccaggcaaagaaaaggcaggataggcacgtggatgaaatccatc

SEQ ID NO: 364 - DNA, 67 bp, Homo sapiens
  source 1..67: mol_type = other DNA
aggaacattttgctaaacaactttcaacagtttaaaaggcaggataggcacgtggatgaaatccatc

SEQ ID NO: 365 - DNA, 67 bp, Homo sapiens
  source 1..67: mol_type = other DNA
ggatagccaccctcagaaccgccaccctcagagaaaaggcaggataggcacgtggatgaaatccatc

SEQ ID NO: 366 - DNA, 67 bp, Homo sapiens
  source 1..67: mol_type = other DNA
aagaaaattcatttcaattacctgagcaaaagaaaaaggcaggataggcacgtggatgaaatccatc

SEQ ID NO: 367 - DNA, 67 bp, Homo sapiens
  source 1..67: mol_type = other DNA
agcagatgaaatagcaatagctatcttaccgaaaaaaggcaggataggcacgtggatgaaatccatc

SEQ ID NO: 368 - DNA, 67 bp, Homo sapiens
  source 1..67: mol_type = other DNA
gtctgagttaagacgctgagaagagtcaatagtaaaaggcaggataggcacgtggatgaaatccatc

SEQ ID NO: 369 - DNA, 67 bp, Homo sapiens
  source 1..67: mol_type = other DNA
agcgggcaaagccggcgaacgtggcgagaaaggaaaaggcaggataggcacgtggatgaaatccatc

SEQ ID NO: 370 - DNA, 67 bp, Homo sapiens
  source 1..67: mol_type = other DNA
agtgtttgattaaagggattttagacaggaacgaaaaggcaggataggcacgtggatgaaatccatc

SEQ ID NO: 371 - DNA, 67 bp, Homo sapiens
  source 1..67: mol_type = other DNA
tattcataatgtttagactggatagcgtccaataaaaagggatgcgaagcgtaggaactgagcagca

SEQ ID NO: 372 - DNA, 67 bp, Homo sapiens
  source 1..67: mol_type = other DNA
aggattatcgagcttcaaagcgaaccagaccggaaaaagggatgcgaagcgtaggaactgagcagca

SEQ ID NO: 373 - DNA, 67 bp, Homo sapiens
  source 1..67: mol_type = other DNA
tgcgcaacttctggtgccggaaaccaggcaaagaaaaagggatgcgaagcgtaggaactgagcagca

SEQ ID NO: 374 - DNA, 67 bp, Homo sapiens
  source 1..67: mol_type = other DNA
aggaacattttgctaaacaactttcaacagtttaaaaagggatgcgaagcgtaggaactgagcagca

SEQ ID NO: 375 - DNA, 67 bp, Homo sapiens
  source 1..67: mol_type = other DNA
ggatagccaccctcagaaccgccaccctcagagaaaaagggatgcgaagcgtaggaactgagcagca

SEQ ID NO: 376 - DNA, 67 bp, Homo sapiens
  source 1..67: mol_type = other DNA
aagaaaattcatttcaattacctgagcaaaagaaaaaagggatgcgaagcgtaggaactgagcagca

SEQ ID NO: 377 - DNA, 67 bp, Homo sapiens
  source 1..67: mol_type = other DNA
agcagatgaaatagcaatagctatcttaccgaaaaaaagggatgcgaagcgtaggaactgagcagca

SEQ ID NO: 378 - DNA, 67 bp, Homo sapiens
  source 1..67: mol_type = other DNA
gtctgagttaagacgctgagaagagtcaatagtaaaaagggatgcgaagcgtaggaactgagcagca

SEQ ID NO: 379 - DNA, 67 bp, Homo sapiens
  source 1..67: mol_type = other DNA
agcgggcaaagccggcgaacgtggcgagaaaggaaaaagggatgcgaagcgtaggaactgagcagca

SEQ ID NO: 380 - DNA, 67 bp, Homo sapiens
  source 1..67: mol_type = other DNA
agtgtttgattaaagggattttagacaggaacgaaaaagggatgcgaagcgtaggaactgagcagca

SEQ ID NO: 381 - DNA, 67 bp, Homo sapiens
  source 1..67: mol_type = other DNA
tattcataatgtttagactggatagcgtccaataaaacgaggtcagtgaacagcagcaagtcctccc

SEQ ID NO: 382 - DNA, 67 bp, Homo sapiens
  source 1..67: mol_type = other DNA
aggattatcgagcttcaaagcgaaccagaccggaaaacgaggtcagtgaacagcagcaagtcctccc

SEQ ID NO: 383 - DNA, 67 bp, Homo sapiens
  source 1..67: mol_type = other DNA
tgcgcaacttctggtgccggaaaccaggcaaagaaaacgaggtcagtgaacagcagcaagtcctccc

SEQ ID NO: 384 - DNA, 67 bp, Homo sapiens
  source 1..67: mol_type = other DNA
aggaacattttgctaaacaactttcaacagtttaaaacgaggtcagtgaacagcagcaagtcctccc

SEQ ID NO: 385 - DNA, 67 bp, Homo sapiens
  source 1..67: mol_type = other DNA
ggatagccaccctcagaaccgccaccctcagagaaaacgaggtcagtgaacagcagcaagtcctccc

SEQ ID NO: 386 - DNA, 67 bp, Homo sapiens
  source 1..67: mol_type = other DNA
aagaaaattcatttcaattacctgagcaaaagaaaaacgaggtcagtgaacagcagcaagtcctccc

SEQ ID NO: 387 - DNA, 67 bp, Homo sapiens
  source 1..67: mol_type = other DNA
agcagatgaaatagcaatagctatcttaccgaaaaaacgaggtcagtgaacagcagcaagtcctccc

SEQ ID NO: 388 - DNA, 67 bp, Homo sapiens
  source 1..67: mol_type = other DNA
gtctgagttaagacgctgagaagagtcaatagtaaaacgaggtcagtgaacagcagcaagtcctccc

SEQ ID NO: 389 - DNA, 67 bp, Homo sapiens
  source 1..67: mol_type = other DNA
agcgggcaaagccggcgaacgtggcgagaaaggaaaacgaggtcagtgaacagcagcaagtcctccc

SEQ ID NO: 390 - DNA, 67 bp, Homo sapiens
  source 1..67: mol_type = other DNA
agtgtttgattaaagggattttagacaggaacgaaaacgaggtcagtgaacagcagcaagtcctccc

SEQ ID NO: 391 - DNA, 67 bp, Homo sapiens
  source 1..67: mol_type = other DNA
tattcataatgtttagactggatagcgtccaataaaagcagtgcgtagtaggagagacgaacgggca

SEQ ID NO: 392 - DNA, 67 bp, Homo sapiens
  source 1..67: mol_type = other DNA
aggattatcgagcttcaaagcgaaccagaccggaaaagcagtgcgtagtaggagagacgaacgggca

SEQ ID NO: 393 - DNA, 67 bp, Homo sapiens
  source 1..67: mol_type = other DNA
tgcgcaacttctggtgccggaaaccaggcaaagaaaagcagtgcgtagtaggagagacgaacgggca

SEQ ID NO: 394 - DNA, 67 bp, Homo sapiens
  source 1..67: mol_type = other DNA
aggaacattttgctaaacaactttcaacagtttaaaagcagtgcgtagtaggagagacgaacgggca

SEQ ID NO: 395 - DNA, 67 bp, Homo sapiens
  source 1..67: mol_type = other DNA
ggatagccaccctcagaaccgccaccctcagagaaaagcagtgcgtagtaggagagacgaacgggca

SEQ ID NO: 396 - DNA, 67 bp, Homo sapiens
  source 1..67: mol_type = other DNA
aagaaaattcatttcaattacctgagcaaaagaaaaagcagtgcgtagtaggagagacgaacgggca

SEQ ID NO: 397 - DNA, 67 bp, Homo sapiens
  source 1..67: mol_type = other DNA
agcagatgaaatagcaatagctatcttaccgaaaaaagcagtgcgtagtaggagagacgaacgggca

SEQ ID NO: 398 - DNA, 67 bp, Homo sapiens
  source 1..67: mol_type = other DNA
gtctgagttaagacgctgagaagagtcaatagtaaaagcagtgcgtagtaggagagacgaacgggca

SEQ ID NO: 399 - DNA, 67 bp, Homo sapiens
  source 1..67: mol_type = other DNA
agcgggcaaagccggcgaacgtggcgagaaaggaaaagcagtgcgtagtaggagagacgaacgggca

SEQ ID NO: 400 - DNA, 67 bp, Homo sapiens
  source 1..67: mol_type = other DNA
agtgtttgattaaagggattttagacaggaacgaaaagcagtgcgtagtaggagagacgaacgggca

SEQ ID NO: 401 - DNA, 67 bp, Homo sapiens
  source 1..67: mol_type = other DNA
tattcataatgtttagactggatagcgtccaataaaacactgtgtgaaggaagacagagagtgggag

SEQ ID NO: 402 - DNA, 67 bp, Homo sapiens
  source 1..67: mol_type = other DNA
aggattatcgagcttcaaagcgaaccagaccggaaaacactgtgtgaaggaagacagagagtgggag

SEQ ID NO: 403 - DNA, 67 bp, Homo sapiens
  source 1..67: mol_type = other DNA
tgcgcaacttctggtgccggaaaccaggcaaagaaaacactgtgtgaaggaagacagagagtgggag

SEQ ID NO: 404 - DNA, 67 bp, Homo sapiens
  source 1..67: mol_type = other DNA
aggaacattttgctaaacaactttcaacagtttaaaacactgtgtgaaggaagacagagagtgggag

SEQ ID NO: 405 - DNA, 67 bp, Homo sapiens
  source 1..67: mol_type = other DNA
ggatagccaccctcagaaccgccaccctcagagaaaacactgtgtgaaggaagacagagagtgggag

SEQ ID NO: 406 - DNA, 67 bp, Homo sapiens
  source 1..67: mol_type = other DNA
aagaaaattcatttcaattacctgagcaaaagaaaaacactgtgtgaaggaagacagagagtgggag

SEQ ID NO: 407 - DNA, 67 bp, Homo sapiens
  source 1..67: mol_type = other DNA
agcagatgaaatagcaatagctatcttaccgaaaaaacactgtgtgaaggaagacagagagtgggag

SEQ ID NO: 408 - DNA, 67 bp, Homo sapiens
  source 1..67: mol_type = other DNA
gtctgagttaagacgctgagaagagtcaatagtaaaacactgtgtgaaggaagacagagagtgggag

SEQ ID NO: 409 - DNA, 67 bp, Homo sapiens
  source 1..67: mol_type = other DNA
agcgggcaaagccggcgaacgtggcgagaaaggaaaacactgtgtgaaggaagacagagagtgggag

SEQ ID NO: 410 - DNA, 67 bp, Homo sapiens
  source 1..67: mol_type = other DNA
agtgtttgattaaagggattttagacaggaacgaaaacactgtgtgaaggaagacagagagtgggag

SEQ ID NO: 411 - DNA, 67 bp, Homo sapiens
  source 1..67: mol_type = other DNA
tattcataatgtttagactggatagcgtccaataaaaagggcatagttgtcctcaaagagctgggtg

SEQ ID NO: 412 - DNA, 67 bp, Homo sapiens
  source 1..67: mol_type = other DNA
aggattatcgagcttcaaagcgaaccagaccggaaaaagggcatagttgtcctcaaagagctgggtg

SEQ ID NO: 413 - DNA, 67 bp, Homo sapiens
  source 1..67: mol_type = other DNA
tgcgcaacttctggtgccggaaaccaggcaaagaaaaagggcatagttgtcctcaaagagctgggtg

SEQ ID NO: 414 - DNA, 67 bp, Homo sapiens
  source 1..67: mol_type = other DNA
aggaacattttgctaaacaactttcaacagtttaaaaagggcatagttgtcctcaaagagctgggtg

SEQ ID NO: 415 - DNA, 67 bp, Homo sapiens
  source 1..67: mol_type = other DNA
ggatagccaccctcagaaccgccaccctcagagaaaaagggcatagttgtcctcaaagagctgggtg

SEQ ID NO: 416 - DNA, 67 bp, Homo sapiens
  source 1..67: mol_type = other DNA
aagaaaattcatttcaattacctgagcaaaagaaaaaagggcatagttgtcctcaaagagctgggtg

SEQ ID NO: 417 - DNA, 67 bp, Homo sapiens
  source 1..67: mol_type = other DNA
agcagatgaaatagcaatagctatcttaccgaaaaaaagggcatagttgtcctcaaagagctgggtg

SEQ ID NO: 418 - DNA, 67 bp, Homo sapiens
  source 1..67: mol_type = other DNA
gtctgagttaagacgctgagaagagtcaatagtaaaaagggcatagttgtcctcaaagagctgggtg

SEQ ID NO: 419 - DNA, 67 bp, Homo sapiens
  source 1..67: mol_type = other DNA
agcgggcaaagccggcgaacgtggcgagaaaggaaaaagggcatagttgtcctcaaagagctgggtg

SEQ ID NO: 420 - DNA, 67 bp, Homo sapiens
  source 1..67: mol_type = other DNA
agtgtttgattaaagggattttagacaggaacgaaaaagggcatagttgtcctcaaagagctgggtg

SEQ ID NO: 421 - DNA, 67 bp, Homo sapiens
  source 1..67: mol_type = other DNA
tattcataatgtttagactggatagcgtccaataaaaccacaacagtacatgtcactctcatcactg

SEQ ID NO: 422 - DNA, 67 bp, Homo sapiens
  source 1..67: mol_type = other DNA
aggattatcgagcttcaaagcgaaccagaccggaaaaccacaacagtacatgtcactctcatcactg

SEQ ID NO: 423 - DNA, 67 bp, Homo sapiens
  source 1..67: mol_type = other DNA
tgcgcaacttctggtgccggaaaccaggcaaagaaaaccacaacagtacatgtcactctcatcactg

SEQ ID NO: 424 - DNA, 67 bp, Homo sapiens
  source 1..67: mol_type = other DNA
aggaacattttgctaaacaactttcaacagtttaaaaccacaacagtacatgtcactctcatcactg

SEQ ID NO: 425 - DNA, 67 bp, Homo sapiens
  source 1..67: mol_type = other DNA
ggatagccaccctcagaaccgccaccctcagagaaaaccacaacagtacatgtcactctcatcactg

SEQ ID NO: 426 - DNA, 67 bp, Homo sapiens
  source 1..67: mol_type = other DNA
aagaaaattcatttcaattacctgagcaaaagaaaaaccacaacagtacatgtcactctcatcactg

SEQ ID NO: 427 - DNA, 67 bp, Homo sapiens
  source 1..67: mol_type = other DNA
agcagatgaaatagcaatagctatcttaccgaaaaaaccacaacagtacatgtcactctcatcactg

SEQ ID NO: 428 - DNA, 67 bp, Homo sapiens
  source 1..67: mol_type = other DNA
gtctgagttaagacgctgagaagagtcaatagtaaaaccacaacagtacatgtcactctcatcactg

SEQ ID NO: 429 - DNA, 67 bp, Homo sapiens
  source 1..67: mol_type = other DNA
agcgggcaaagccggcgaacgtggcgagaaaggaaaaccacaacagtacatgtcactctcatcactg

SEQ ID NO: 430 - DNA, 67 bp, Homo sapiens
  source 1..67: mol_type = other DNA
agtgtttgattaaagggattttagacaggaacgaaaaccacaacagtacatgtcactctcatcactg

SEQ ID NO: 431 - DNA, 67 bp, Homo sapiens
  source 1..67: mol_type = other DNA
tattcataatgtttagactggatagcgtccaataaaaagttctagaccccatgtaataaaaggtggt

SEQ ID NO: 432 - DNA, 67 bp, Homo sapiens
  source 1..67: mol_type = other DNA
aggattatcgagcttcaaagcgaaccagaccggaaaaagttctagaccccatgtaataaaaggtggt

SEQ ID NO: 433 - DNA, 67 bp, Homo sapiens
  source 1..67: mol_type = other DNA
tgcgcaacttctggtgccggaaaccaggcaaagaaaaagttctagaccccatgtaataaaaggtggt

SEQ ID NO: 434 - DNA, 67 bp, Homo sapiens
  source 1..67: mol_type = other DNA
aggaacattttgctaaacaactttcaacagtttaaaaagttctagaccccatgtaataaaaggtggt

SEQ ID NO: 435 - DNA, 67 bp, Homo sapiens
  source 1..67: mol_type = other DNA
ggatagccaccctcagaaccgccaccctcagagaaaaagttctagaccccatgtaataaaaggtggt

SEQ ID NO: 436 - DNA, 67 bp, Homo sapiens
  source 1..67: mol_type = other DNA
aagaaaattcatttcaattacctgagcaaaagaaaaaagttctagaccccatgtaataaaaggtggt

SEQ ID NO: 437 - DNA, 67 bp, Homo sapiens
  source 1..67: mol_type = other DNA
agcagatgaaatagcaatagctatcttaccgaaaaaaagttctagaccccatgtaataaaaggtggt

SEQ ID NO: 438 - DNA, 67 bp, Homo sapiens
  source 1..67: mol_type = other DNA
gtctgagttaagacgctgagaagagtcaatagtaaaaagttctagaccccatgtaataaaaggtggt

SEQ ID NO: 439 - DNA, 67 bp, Homo sapiens
  source 1..67: mol_type = other DNA
agcgggcaaagccggcgaacgtggcgagaaaggaaaaagttctagaccccatgtaataaaaggtggt

SEQ ID NO: 440 - DNA, 67 bp, Homo sapiens
  source 1..67: mol_type = other DNA
agtgtttgattaaagggattttagacaggaacgaaaaagttctagaccccatgtaataaaaggtggt

SEQ ID NO: 441 - DNA, 67 bp, Homo sapiens
  source 1..67: mol_type = other DNA
tattcataatgtttagactggatagcgtccaataaaattccaatgtgtatggtacagtttccattgt

SEQ ID NO: 442 - DNA, 67 bp, Homo sapiens
  source 1..67: mol_type = other DNA
aggattatcgagcttcaaagcgaaccagaccggaaaattccaatgtgtatggtacagtttccattgt

SEQ ID NO: 443 - DNA, 67 bp, Homo sapiens
  source 1..67: mol_type = other DNA
tgcgcaacttctggtgccggaaaccaggcaaagaaaattccaatgtgtatggtacagtttccattgt

SEQ ID NO: 444 - DNA, 67 bp, Homo sapiens
  source 1..67: mol_type = other DNA
aggaacattttgctaaacaactttcaacagtttaaaattccaatgtgtatggtacagtttccattgt

SEQ ID NO: 445 - DNA, 67 bp, Homo sapiens
  source 1..67: mol_type = other DNA
ggatagccaccctcagaaccgccaccctcagagaaaattccaatgtgtatggtacagtttccattgt

SEQ ID NO: 446 - DNA, 67 bp, Homo sapiens
  source 1..67: mol_type = other DNA
aagaaaattcatttcaattacctgagcaaaagaaaaattccaatgtgtatggtacagtttccattgt

SEQ ID NO: 447 - DNA, 67 bp, Homo sapiens
  source 1..67: mol_type = other DNA
agcagatgaaatagcaatagctatcttaccgaaaaaattccaatgtgtatggtacagtttccattgt

SEQ ID NO: 448 - DNA, 67 bp, Homo sapiens
  source 1..67: mol_type = other DNA
gtctgagttaagacgctgagaagagtcaatagtaaaattccaatgtgtatggtacagtttccattgt

SEQ ID NO: 449 - DNA, 67 bp, Homo sapiens
  source 1..67: mol_type = other DNA
agcgggcaaagccggcgaacgtggcgagaaaggaaaattccaatgtgtatggtacagtttccattgt

SEQ ID NO: 450 - DNA, 67 bp, Homo sapiens
  source 1..67: mol_type = other DNA
agtgtttgattaaagggattttagacaggaacgaaaattccaatgtgtatggtacagtttccattgt

SEQ ID NO: 451 - DNA, 67 bp, Homo sapiens
  source 1..67: mol_type = other DNA
tattcataatgtttagactggatagcgtccaataaaagtctttgaagagccggcttctctaaacagg

SEQ ID NO: 452 - DNA, 67 bp, Homo sapiens
  source 1..67: mol_type = other DNA
aggattatcgagcttcaaagcgaaccagaccggaaaagtctttgaagagccggcttctctaaacagg

SEQ ID NO: 453 - DNA, 67 bp, Homo sapiens
  source 1..67: mol_type = other DNA
tgcgcaacttctggtgccggaaaccaggcaaagaaaagtctttgaagagccggcttctctaaacagg

SEQ ID NO: 454 - DNA, 67 bp, Homo sapiens
  source 1..67: mol_type = other DNA
aggaacattttgctaaacaactttcaacagtttaaaagtctttgaagagccggcttctctaaacagg

SEQ ID NO: 455 - DNA, 67 bp, Homo sapiens
  source 1..67: mol_type = other DNA
ggatagccaccctcagaaccgccaccctcagagaaaagtctttgaagagccggcttctctaaacagg

SEQ ID NO: 456 - DNA, 67 bp, Homo sapiens
  source 1..67: mol_type = other DNA
aagaaaattcatttcaattacctgagcaaaagaaaaagtctttgaagagccggcttctctaaacagg

SEQ ID NO: 457 - DNA, 67 bp, Homo sapiens
  source 1..67: mol_type = other DNA
agcagatgaaatagcaatagctatcttaccgaaaaaagtctttgaagagccggcttctctaaacagg

SEQ ID NO: 458 - DNA, 67 bp, Homo sapiens
  source 1..67: mol_type = other DNA
gtctgagttaagacgctgagaagagtcaatagtaaaagtctttgaagagccggcttctctaaacagg

SEQ ID NO: 459 - DNA, 67 bp, Homo sapiens
  source 1..67: mol_type = other DNA
agcgggcaaagccggcgaacgtggcgagaaaggaaaagtctttgaagagccggcttctctaaacagg

SEQ ID NO: 460 - DNA, 67 bp, Homo sapiens
  source 1..67: mol_type = other DNA
agtgtttgattaaagggattttagacaggaacgaaaagtctttgaagagccggcttctctaaacagg

SEQ ID NO: 461 - DNA, 67 bp, Homo sapiens
  source 1..67: mol_type = other DNA
tattcataatgtttagactggatagcgtccaataaaaagccacaaacaacgccaatccagtatcact

SEQ ID NO: 462 - DNA, 67 bp, Homo sapiens
  source 1..67: mol_type = other DNA
aggattatcgagcttcaaagcgaaccagaccggaaaaagccacaaacaacgccaatccagtatcact

SEQ ID NO: 463 - DNA, 67 bp, Homo sapiens
  source 1..67: mol_type = other DNA
tgcgcaacttctggtgccggaaaccaggcaaagaaaaagccacaaacaacgccaatccagtatcact

SEQ ID NO: 464 - DNA, 67 bp, Homo sapiens
  source 1..67: mol_type = other DNA
aggaacattttgctaaacaactttcaacagtttaaaaagccacaaacaacgccaatccagtatcact

SEQ ID NO: 465 - DNA, 67 bp, Homo sapiens
  source 1..67: mol_type = other DNA
ggatagccaccctcagaaccgccaccctcagagaaaaagccacaaacaacgccaatccagtatcact

SEQ ID NO: 466 - DNA, 67 bp, Homo sapiens
  source 1..67: mol_type = other DNA
aagaaaattcatttcaattacctgagcaaaagaaaaaagccacaaacaacgccaatccagtatcact

SEQ ID NO: 467 - DNA, 67 bp, Homo sapiens
  source 1..67: mol_type = other DNA
agcagatgaaatagcaatagctatcttaccgaaaaaaagccacaaacaacgccaatccagtatcact

SEQ ID NO: 468 - DNA, 67 bp, Homo sapiens
  source 1..67: mol_type = other DNA
gtctgagttaagacgctgagaagagtcaatagtaaaaagccacaaacaacgccaatccagtatcact

SEQ ID NO: 469 - DNA, 67 bp, Homo sapiens
  source 1..67: mol_type = other DNA
agcgggcaaagccggcgaacgtggcgagaaaggaaaaagccacaaacaacgccaatccagtatcact

SEQ ID NO: 470 - DNA, 67 bp, Homo sapiens
  source 1..67: mol_type = other DNA
agtgtttgattaaagggattttagacaggaacgaaaaagccacaaacaacgccaatccagtatcact

SEQ ID NO: 471 - DNA, 67 bp, Homo sapiens
  source 1..67: mol_type = other DNA
tattcataatgtttagactggatagcgtccaataaaatcactaaaagagggccccaatactacaaaa

SEQ ID NO: 472 - DNA, 67 bp, Homo sapiens
  source 1..67: mol_type = other DNA
aggattatcgagcttcaaagcgaaccagaccggaaaatcactaaaagagggccccaatactacaaaa

SEQ ID NO: 473 - DNA, 67 bp, Homo sapiens
  source 1..67: mol_type = other DNA
tgcgcaacttctggtgccggaaaccaggcaaagaaaatcactaaaagagggccccaatactacaaaa

SEQ ID NO: 474 - DNA, 67 bp, Homo sapiens
  source 1..67: mol_type = other DNA
aggaacattttgctaaacaactttcaacagtttaaaatcactaaaagagggccccaatactacaaaa

SEQ ID NO: 475 - DNA, 67 bp, Homo sapiens
  source 1..67: mol_type = other DNA
ggatagccaccctcagaaccgccaccctcagagaaaatcactaaaagagggccccaatactacaaaa

SEQ ID NO: 476 - DNA, 67 bp, Homo sapiens
  source 1..67: mol_type = other DNA
aagaaaattcatttcaattacctgagcaaaagaaaaatcactaaaagagggccccaatactacaaaa

SEQ ID NO: 477 - DNA, 67 bp, Homo sapiens
  source 1..67: mol_type = other DNA
agcagatgaaatagcaatagctatcttaccgaaaaaatcactaaaagagggccccaatactacaaaa

SEQ ID NO: 478 - DNA, 67 bp, Homo sapiens
  source 1..67: mol_type = other DNA
gtctgagttaagacgctgagaagagtcaatagtaaaatcactaaaagagggccccaatactacaaaa

SEQ ID NO: 479 - DNA, 67 bp, Homo sapiens
  source 1..67: mol_type = other DNA
agcgggcaaagccggcgaacgtggcgagaaaggaaaatcactaaaagagggccccaatactacaaaa

SEQ ID NO: 480 - DNA, 67 bp, Homo sapiens
  source 1..67: mol_type = other DNA
agtgtttgattaaagggattttagacaggaacgaaaatcactaaaagagggccccaatactacaaaa

SEQ ID NO: 481 - DNA, 67 bp, Homo sapiens
  source 1..67: mol_type = other DNA
tattcataatgtttagactggatagcgtccaataaaaacaaaaaccaatggctctttttcttccgga

SEQ ID NO: 482 - DNA, 67 bp, Homo sapiens
  source 1..67: mol_type = other DNA
aggattatcgagcttcaaagcgaaccagaccggaaaaacaaaaaccaatggctctttttcttccgga

SEQ ID NO: 483 - DNA, 67 bp, Homo sapiens
  source 1..67: mol_type = other DNA
tgcgcaacttctggtgccggaaaccaggcaaagaaaaacaaaaaccaatggctctttttcttccgga

SEQ ID NO: 484 - DNA, 67 bp, Homo sapiens
  source 1..67: mol_type = other DNA
aggaacattttgctaaacaactttcaacagtttaaaaacaaaaaccaatggctctttttcttccgga

SEQ ID NO: 485 - DNA, 67 bp, Homo sapiens
  source 1..67: mol_type = other DNA
ggatagccaccctcagaaccgccaccctcagagaaaaacaaaaaccaatggctctttttcttccgga

SEQ ID NO: 486 - DNA, 67 bp, Homo sapiens
  source 1..67: mol_type = other DNA
aagaaaattcatttcaattacctgagcaaaagaaaaaacaaaaaccaatggctctttttcttccgga

SEQ ID NO: 487 - DNA, 67 bp, Homo sapiens
  source 1..67: mol_type = other DNA
agcagatgaaatagcaatagctatcttaccgaaaaaaacaaaaaccaatggctctttttcttccgga

SEQ ID NO: 488 - DNA, 67 bp, Homo sapiens
  source 1..67: mol_type = other DNA
gtctgagttaagacgctgagaagagtcaatagtaaaaacaaaaaccaatggctctttttcttccgga

SEQ ID NO: 489 - DNA, 67 bp, Homo sapiens
  source 1..67: mol_type = other DNA
agcgggcaaagccggcgaacgtggcgagaaaggaaaaacaaaaaccaatggctctttttcttccgga

SEQ ID NO: 490 - DNA, 67 bp, Homo sapiens
  source 1..67: mol_type = other DNA
agtgtttgattaaagggattttagacaggaacgaaaaacaaaaaccaatggctctttttcttccgga